European Patent Specification EP 3 833 786 B1, published December 27, 2023. Title: Recombinant nucleic acid construct. Applicant: Pantherna Therapeutics GmbH. The sequence listing filed with the application follows.

SEQUENCE LISTING (125 sequences)

SEQ ID NO: 1 - DNA, 38 bp, Artificial Sequence
  Synthetic
taatacgactcactatagggccctaagccatcagcaat

SEQ ID NO: 2 - DNA, 38 bp, Artificial Sequence
  Synthetic
taatacgactcactataggaaagtgattgattcggata

SEQ ID NO: 3 - DNA, 38 bp, Artificial Sequence
  Synthetic
taatacgactcactataggtccccattgaataacagcc

SEQ ID NO: 4 - DNA, 38 bp, Artificial Sequence
  Synthetic
taatacgactcactataggataaaagcccaggggcaag

SEQ ID NO: 5 - DNA, 38 bp, Artificial Sequence
  Synthetic
taatacgactcactatagggtcagccatctttcaattg

SEQ ID NO: 6 - DNA, 38 bp, Artificial Sequence
  Synthetic
taatacgactcactataggcatatcttcattcttcact

SEQ ID NO: 7 - DNA, 38 bp, Artificial Sequence
  Synthetic
taatacgactcactataggataaaagcctagtggccat

SEQ ID NO: 8 - DNA, 38 bp, Artificial Sequence
  Synthetic
taatacgactcactatagggaggaaccgagaggctgag

SEQ ID NO: 9 - DNA, 38 bp, Artificial Sequence
  Synthetic
taatacgactcactataggggagctgtttacccccact

SEQ ID NO: 10 - DNA, 38 bp, Artificial Sequence; identical to SEQ ID NO: 2
  Synthetic

SEQ ID NO: 11 - DNA, 139 bp, Artificial Sequence
  Synthetic
ttttttttttttttttttttttttttttttttttttttttttttttttttttttttttttttttttttttttttttttttttttttttttttttttttttttttttttttttttttttttgccttttgcaagataagag

SEQ ID NO: 12 - DNA, 139 bp, Artificial Sequence; identical to SEQ ID NO: 11
  Synthetic

SEQ ID NO: 13 - DNA, 139 bp, Artificial Sequence
  Synthetic
ttttttttttttttttttttttttttttttttttttttttttttttttttttttttttttttttttttttttttttttttttttttttttttttttttttttttttttttttttttttttgaattttaaagtttattta

SEQ ID NO: 14 - DNA, 139 bp, Artificial Sequence
  Synthetic
ttttttttttttttttttttttttttttttttttttttttttttttttttttttttttttttttttttttttttttttttttttttttttttttttttttttttttttttttttttttttatagtttaatgtattttaa

SEQ ID NO: 15 - DNA, 139 bp, Artificial Sequence
  Synthetic
ttttttttttttttttttttttttttttttttttttttttttttttttttttttttttttttttttttttttttttttttttttttttttttttttttttttttttttttttttttttttttaactacatctaaaccca

SEQ ID NO: 16 - DNA, 139 bp, Artificial Sequence
  Synthetic
tttttttttttttttttttttttttttttttttttttttttttttttttttttttttttttttttttttttttttttttttttttttttttttttttttttttttttttttttttttttttcgctacaaatcaaaaggc

SEQ ID NO: 17 - DNA, 139 bp, Artificial Sequence
  Synthetic
tttttttttttttttttttttttttttttttttttttttttttttttttttttttttttttttttttttttttttttttttttttttttttttttttttttttttttttttttttttttttgtacaaaaatatatttat

SEQ ID NO: 18 - DNA, 144 bp, Artificial Sequence
  Synthetic
tttttttttttttttttttttttttttttttttttttttttttttttttttttttttttttttttttttttttttttttttttttttttttttttttttttttttttttttttttttttttttacagtaaggaaaaaaatattt

SEQ ID NO: 19 - DNA, 139 bp, Artificial Sequence; identical to SEQ ID NO: 11
  Synthetic

SEQ ID NO: 20 - DNA, 73 bp, Homo sapiens
  5'UTR (1)..(73)
gaggaaccgagaggctgagactaacccagaaacatccaattctcaaactgaagctcgcactctcgcctccagc

SEQ ID NO: 21 - DNA, 69 bp, Homo sapiens
  sig_peptide (1)..(69)
atgaaagtctctgccgcccttctgtgcctgctgctcatagcagccaccttcattccccaagggctcgct

SEQ ID NO: 22 - protein, 23 aa, Homo sapiens
  SIGNAL (1)..(23)
MKVSAALLCLLLIAATFIPQGLA

SEQ ID NO: 23 - DNA, 373 bp, Homo sapiens
  3'UTR (1)..(373)
acactcactccacaacccaagaatctgcagctaacttattttcccctagctttccccagacaccctgttttattttattataatgaattttgtttgttgatgtgaaacattatgccttaagtaatgttaattcttatttaagttattgatgttttaagtttatctttcatggtactagtgttttttagatacagagacttggggaaattgcttttcctcttgaaccacagttctacccctgggatgttttgagggtctttgcaagaatcattaatacaaagaattttttttaacattccaatgcattgctaaaatattattgtggaaatgaatattttgtaactattacaccaaataaatatatttttgtaca

SEQ ID NO: 24 - DNA, 94 bp, Spinacia oleracea
  5'UTR (1)..(94)
catatcttcattcttcactctttccccccccccccttatcctcctatctaatcctctcatctctctcctcctcttcctccaacaacaactaaca

SEQ ID NO: 25 - DNA, 148 bp, Spinacia oleracea
  3'UTR (1)..(148)
ttttgagtaattttcaattttgtttttgtttttgtttttgttgttgggagttgttgtaatttggtaaatgttggggtcactaaaatcttttgttgcaattttagcacctttttattagatatataaaattgggtttagatgtagttaa

SEQ ID NO: 26 - DNA, 329 bp, Homo sapiens
  5'UTR (1)..(329)
aaagtgattgattcggatactgacactgtaggatctggggagagaggaacaaaggaccgtgaaagctgctctgtaaaagctgacacagccctcccaagtgagcaggactgttcttcccactgcaatctgacagtttactgcatgcctggagagaacacagcagtaaaaaccaggtttgctactggaaaaagaggaaagagaagactttcattgacggacccagccatggcagcgtagcagccctgcgttttagacggcagcagctcgggactctggacgtgtgtttgccctcaagtttgctaagctgctggtttattactgaagaaaga

SEQ ID NO: 27 - DNA, 54 bp, Homo sapiens
  sig_peptide (1)..(54)
atgtggcagattgttttctttactctgagctgtgatcttgtcttggccgcagcc

SEQ ID NO: 28 - protein, 18 aa, Homo sapiens
  SIGNAL (1)..(18)
MWQIVFFTLSCDLVLAAA

SEQ ID NO: 29 - DNA, 3450 bp, Homo sapiens
  3'UTR (1)..(3450)
acatcccagtccacctgaggaactgtctcgaactattttcaaagacttaagcccagtgcactgaaagtcacggctgcgcactgtgtcctcttccaccacagagggcgtgtgctcggtgctgacgggacccacatgctccagattagagcctgtaaactttatcacttaaacttgcatcacttaacggaccaaagcaagaccctaaacatccataattgtgattagacagaacacctatgcaaagatgaacccgaggctgagaatcagactgacagtttacagacgctgctgtcacaaccaagaatgttatgtgcaagtttatcagtaaataactggaaaacagaacacttatgttatacaatacagatcatcttggaactgcattcttctgagcactgtttatacactgtgtaaatacccatatgtcctgaattcaccatcactatcacaattaaaaggaagaaaaaaactctctaagccataaaaagacatattcagggatattctgagaaggggttactagaagtttaatatttggaaaaacagttagtgcatttttactccatctcttaggtgctttaaatttttatttcaaaaacagcgtatttacatttatgttgacagcttagttataagttaatgctcaaatacgtatttcaaatttatatggtagaaacttccagaatctctgaaattatcaacagaaacgtgccattttagtttatatgcagaccgtactatttttttctgcctgattgttaaatatgaaggtatttttagtaattaaatataacttattaggggatatgcctatgtttaacttttatgataatatttacaattttataatttgtttccaaaagacctaattgtgccttgtgataaggaaacttcttacttttaatgatgaggaaaattatacatttcattctatgacaaagaaactttactatcttctcactattctaaaacagaggtctgttttctttcctagtaagatatatttttatagaactagactacaatttaatttctggttgagaaaagccttctatttaagaaatttacaaagctatatgtctcaagattcacccttaaatttacttaaggaaaaaaataattgacactagtaagtttttttatgtcaatcagcaaactgaaaaaaaaaaaagggtttcaaagtgcaaaaacaaaatctgatgttcataatatatttaaatatttaccaaaaatttgagaacacagggctgggcgcagtggctcacacctataatcccagtacattggtaggcaaggtgggcagatcacctgaggtcaggagttcaagaccagcctggacaacatggtgaaaccctgtctctactaaataatacaaaaattagccaggcgtgctggcgggcacctgtaatcccagctactcgggaggctgaggcagggagaattgcttgcaccagggaggtagaggttgcagtgagccaagatcgcaccactgcactccagccggggcaacagagcaagactccatctcaaaaaaaaaaaaaaaaaaagaaagaaaagaaaatttgagaacacagctttatactcgggactacaaaaccataaactcctggagttttaactccttttgaaattttcatagtacaattaatactaatgaacatttgtgtaaagctttataatttaaaggcaatttctcatatattcttttctgaatcatttgcaaggaagttcagagtccagtctgtaactagcatctactatatgtctgtcttcaccttacagtgttctaccattattttttctttattccatttcaaaatctaatttattttaccccaacttctccccaccacttgacgtagttttagaacacacaggtgttgctacatatttggagtcaatgatggactctggcaaagtcaaggctctgttttatttccaccaaggtgcacttttccaacaactatttaactagttaagaacctccctatcttagaactgtatctactttatatttaagaaggttttatgaattcaacaacggtatcatggccttgtatcaagttgaaaaacaactgaaaataagaaaatttcacagcctcgaaagacaacaacaagtttctaggatatctcaatgacaagagtgatggatacttaggtagggaaacgctaatgcaggaaaaactggcaacaacacaatttatatcaattctctttgtaggcaggtgataaaaaattcaaggacaaatctcattatgtcattgtgcatcatatataatctcttatgagcgagaatggggggaatttgtgtttttactttacacttcaattccttacacggtatttcaaacaaacagttttgctgagaggagcttttgtctctccttaagaaaatgtttataaagctgaaaggaaatcaaacagtaatcttaaaaatgaaaacaaaacaacccaacaacctagataactacagtgatcagggagcacagttcaactccttgttatgttttagtcatatggcctactcaaacagctaaataacaacaccagtggcagataaaaatcaccatttatctttcagctattaatcttttgaatgaataaactgtgacaaacaaattaacatttttgaacatgaaaggcaacttctgcacaatcctgtatccaagcaaactttaaattatccacttaattattacttaatcttaaaaaaaattagaacccagaacttttcaatgaagcatttgaaagttgaagtggaatttaggaaagccataaaaatataaatactgttatcacagcaccagcaagccataatctttatacctatcagttctatttctattaacagtaaaaacattaagcaagatataagactacctgcccaagaattcagtcttttttcatttttgtttttctcagttctgaggatgttaatcgtcaaattttctttggactgcattcctcactactttttgcacaatggtctcacgttctcacatttgttctcgcgaataaattgataaaaggtgttaagttctgtgaatgtctttttaattatgggcataattgtgcttgactggataaaaacttaagtccacccttatgtttataataatttcttgagaacagcaaactgcatttaccatcgtaaaacaacatctgacttacgggagctgcagggaagtggtgagacagttcgaacggctcctcagaaatccagtgacccaattctaaagaccatagcacctgcaagtgacacaacaagcagatttattatacatttattagccttagcaggcaataaaccaagaatcactttgaagacacagcaaaaagtgatacactccgcagatctgaaatagatgtgttctcagacaacaaagtcccttcagaatcttcatgttgcataaatgttatgaatattaataaaaagttgattgagaaaaa

SEQ ID NO: 30 - DNA, 121 bp, Homo sapiens
  5'UTR (1)..(121)
gtctcaatattagagtctcaacccccaataaatataggactggagatgtctgaggctcattctgccctcgagcccaccgggaacgaaagagaagctctatctcccctccaggagcccagct

SEQ ID NO: 31 - DNA, 87 bp, Homo sapiens
  sig_peptide (1)..(87)
atgaactccttctccacaagcgccttcggtccagttgccttctccctggggctgctcctggtgttgcctgctgccttccctgcccca

SEQ ID NO: 32 - protein, 29 aa, Homo sapiens
  SIGNAL (1)..(29)
MNSFSTSAFGPVAFSLGLLLVLPAAFPAP

SEQ ID NO: 33 - DNA, 429 bp, Homo sapiens
  3'UTR (1)..(429)
catgggcacctcagattgttgttgttaatgggcattccttcttctggtcagaaacctgtccactgggcacagaacttatgttgttctctatggagaactaaaagtatgagcgttaggacactattttaattatttttaatttattaatatttaaatatgtgaagctgagttaatttatgtaagtcatatttatatttttaagaagtaccacttgaaacattttatgtattagttttgaaataataatggaaagtggctatgcagtttgaatatcctttgtttcagagccagatcatttcttggaaagtgtaggcttacctcaaataaatggctaacttatacatatttttaaagaaatatttatattgtatttatataatgtataaatggtttttataccaataaatggcattttaaaaaattcagcaa

SEQ ID NO: 34 - DNA, 255 bp, Homo sapiens
  5'UTR (1)..(255)
gtggcagctcacagctattgtggtgggaaagggagggtggttggtggatgtcacagcttgggctttatctcccccagcagtggggactccacagcccctgggctacataacagcaagacagtccggagctgtagcagacctgattgagcctttgcagcagctgagagcatggcctagggtgggcggcaccattgtccagcagctgagtttcccagggaccttggagatagccgcagccctcatttgcaggggaag

SEQ ID NO: 35 - DNA, 66 bp, Homo sapiens
  sig_peptide (1)..(66)
atgattcctgccagatttgccggggtgctgcttgctctggccctcattttgccagggaccctttgt

SEQ ID NO: 36 - protein, 22 aa, Homo sapiens
  SIGNAL (1)..(22)
MIPARFAGVLLALALILPGTLC

SEQ ID NO: 37 - DNA, 141 bp, Homo sapiens
  3'UTR (1)..(141)
ggctgctgcagctgcatgggtgcctgctgctgcctgccttggcctgatggccaggccagagtgctgccagtcctctgcatgttctgctcttgtgcccttctgagcccacaataaaggctgagctcttatcttgcaaaaggc

SEQ ID NO: 38 - DNA, 243 bp, Homo sapiens
  5'UTR (1)..(243)
ataaaagcccaggggcaagcggtccggataacggctagcctgaggagctgctgcgacagtccactacctttttcgagagtgactcccgttgtcccaaggcttcccagagcgaacctgtgcggctgcaggcaccggcgcgtcgagtttccggcgtccggaaggaccgagctcttctcgcggatccagtgttccgtttccagcccccaatctcagagcggagccgacagagagcagggaaccggc

SEQ ID NO: 39 - DNA, 258 bp, Homo sapiens
  3'UTR (1)..(258)
gggcctttccaagattgctgtttttgttttggagcttcaagactttgcatttcctagtatttctgtttgtcagttctcaatttcctgtgtttgcaatgttgaaattttttggtgaagtactgaacttgctttttttccggtttctacatgcagagatgaatttatactgccatcttacgactatttcttctttttaatacacttaactcaggccattttttaagttggttacttcaaagtaaataaactttaaaattc

SEQ ID NO: 40 - DNA, 261 bp, Homo sapiens
  5'UTR (1)..(261)
gggctgggggagggtatataagccgagtaggcgacggtgaggtcgacgccggccaagacagcacagacagattgacctattggggtgtttcgcgagtgtgagagggaagcgccgcggcctgtatttctagacctgcccttcgcctggttcgtggcgccttgtgaccccgggcccctgccgcctgcaagtcggaaattgcgctgtgctcctgtgctacggcctgtggctggactgcctgctgctgcccaactggctggcaag

SEQ ID NO: 41 - DNA, 54 bp, Homo sapiens
  sig_peptide (1)..(54)
atgaagctctccctggtggccgcgatgctgctgctgctcagcgcggcgcgggcc

SEQ ID NO: 42 - protein, 18 aa, Homo sapiens
  SIGNAL (1)..(18)
MKLSLVAAMLLLLSAARA

SEQ ID NO: 43 - DNA, 1744 bp, Homo sapiens
  3'UTR (1)..(1744)
acactgatctgctagtgctgtaatattgtaaatactggactcaggaacttttgttaggaaaaaattgaaagaacttaagtctcgaatgtaattggaatcttcacctcagagtggagttgaaactgctatagcctaagcggctgtttactgcttttcattagcagttgctcacatgtctttgggtgggggggagaagaagaattggccatcttaaaaagcgggtaaaaaacctgggttagggtgtgtgttcaccttcaaaatgttctatttaacaactgggtcatgtgcatctggtgtaggaagttttttctaccataagtgacaccaataaatgtttgttatttacactggtctaatgtttgtgagaagcttctaattagatcaattacttattttaggaaatttaagactagatactcgtgtgtggggtgaggggagggagtatttggtatgttgggataaggaaacacttctatttaatgcttccagggatttttttttttttttttaaccctcctgggcccaagtgatccttccacctcagtctcccagctaattgagaccacaggcttgttaccaccatgctcggcttttgcattaatctaagaaaaggggagagaagttaatccacatctttactcaggcaaggggcatttcacagtgcccaagagtggggttttcttgaacatacttggtttcctatttccccttatctttctaaaactgcctttctggtggctttttttaaaattattactaatgatgcttttatagctgcttggattctctgagaaatgatggggagtgagtgatcactggtattaactttatacacttggatttcatttgtaactttaggatgtaaaggtatattgtgaaccctagctgtgtcagaatctccatccctgaaatttctcattagtggtactggggtgggatcttggatggtgacattgaaactacactaaatcccctcactatgaatgggttgttaaaggcaatggtttgtgtcaaaactggtttaggattacttagattgtgttcctgaagaaaagagtccaggtaaatggtatgatcaataaaggacaggctggtgctaacataaaatccaatattgtaatcctagcactttgggaggccaaggcgggtggatcacaaggtcaagagatagagaccatctttgccaacatggtgaaactccatctctactgaaaatacaaaaattagctgggcgtggtagtgcaagctgaaggctgaggcaggagaatcactcgaacccgggaggcagaggttgcagtgagccgagatcacaccactgtactccagcccggcactccagcctggcgacaagagtgagactccacctcaaaaaaaaaaaaaagaatccaatactgcccaaggataggtattttatagatgggcaactggctgaaaggttaattctctagggctagtagaactggatcccaacaccaaactcttaattagacctaggcctcagctgcactgcccgaaaagcatttgggcagaccctgagcagaatactggtctcaggccaagcccaatacagccattaaagatgacctacagtgctgtgtaccctggggcaatagggttaaatggtagttagcaactagggctagtcttcccttacctcaaaggctctcactaccgtggaccacctagtctgtaactctttctgaggagctgttactgaatattaaaaagatagacttcaactatg

SEQ ID NO: 44 - DNA, 128 bp, Homo sapiens
  5'UTR (1)..(128)
gtcagccatctttcaattgtgttcgcagccgccgccgcgccgccgtcgctctccaacgccagcgccgcctctcgctcgccgagctccagccgaaggagaaggggggtaagtaaggaggtctctgtacc

SEQ ID NO: 45 - DNA, 521 bp, Homo sapiens
  3'UTR (1)..(521)
gaatccactatgatgggaaacatttcattctcaaaaaaaaaaaaaaaaatttctcttcttcctgttattggtagttctgaacgttagatattttttttccatggggtcaaaaggtacctaagtatatgattgcgagtggaaaaataggggacagaaatcaggtattggcagtttttccattttcatttgtgtgtgaatttttaatataaatgcggagacgtaaagcattaatgcaagttaaaatgtttcagtgaacaagtttcagcggttcaactttataataattataaataaacctgttaaatttttctggacaatgccagcatttggatttttttaaaacaagtaaatttcttattgatggcaactaaatggtgtttgtagcatttttatcatacagtagattccatccattcactatacttttctaactgagttgtcctacatgcaagtacatgtttttaatgttgtctgtcttctgtgctgttcctgtaagtttgctattaaaatacattaaacta

SEQ ID NO: 46 - DNA, 118 bp, Homo sapiens
  5'UTR (1)..(118)
tccccattgaataacagccaagttgctttggtttctatttctttgttaagtcgttccctctacaaaggacttcctagtgggtgtgaaaggcagcggtggccacagaggcggcggagag

SEQ ID NO: 47 - DNA, 578 bp, Homo sapiens
  3'UTR (1)..(578)
gcggcttcctggccctggggccgggggctggggtgtggggcagtctgggtcctctcatcatccccacttcccaggcccagcctttccaaccctgcctgggatctgggctttaatgcagaggccatgtccttgtctggtcctgcttctggctacagccaccctggaacggagaaggcagctgacggggattgccttcctcagccgcagcagcacctggggctccagctgctggaatcctaccatcccaggaggcaggcacagccagggagaggggaggagtgggcagtgaagatgaagccccatgctcagtcccctcccatcccccacgcagctccaccccagtcccaagccaccagctgtctgctcctggtgggaggtggcctcctcagcccctcctctctgacctttaacctcactctcaccttgcaccgtgcaccaacccttcacccctcctggaaagcaggcctgatggcttcccactggcctccaccacctgaccagagtgttctcttcagaggactggctcctttcccagtgtccttaaaataaagaaatgaaaatgcttgttggcacattca

SEQ ID NO: 48 - DNA, 4367 bp, Artificial Sequence
  Synthetic
gccctaagccatcagcaatccttagtataggggcacactcatgcattcctgtcaagtcatcttgtgaaaggctgcctgcttccagcttggcttggatgtgcaaccttaataaaactcactgaggtctgggagaaaatagcagatctgcagcagatagggtagaggaaagggtctagaatatgtacacgcagctgactcaggcaggctccatgctgaacggtcacacagagaggaaacaataaatctcagctactatgcaataaatatctcaagttttaacgaagaaaaacatcattgcagtgaaataaaaaattttaaaattttagaacaaagctaacaaatggctagttttctatgattcttcttcaaacgctttctttgagggggaaagagtcaaacaaacaagcagttttacctgaaataaagaactagttttagaggtcagaagaaaggagcaagttttgcgagaggcacggaaggagtgtgctggcagtacaatgacagttttcctttcctttgctttcctcgctgccattctgactcacatagggtgcagcaatcagcgccgaagtccagaaaacagtgggagaagatataaccggattcaacatgggcaatgtgcctacactttcattcttccagaacacgatggcaactgtcgtgagagtacgacagaccagtacaacacaaacgctctgcagagagatgctccacacgtggaaccggatttctcttcccagaaacttcaacatctggaacatgtgatggaaaattatactcagtggctgcaaaaacttgagaattacattgtggaaaacatgaagtcggagatggcccagatacagcagaatgcagttcagaaccacacggctaccatgctggagataggaaccagcctcctctctcagactgcagagcagaccagaaagctgacagatgttgagacccaggtactaaatcaaacttctcgacttgagatacagctgctggagaattcattatccacctacaagctagagaagcaacttcttcaacagacaaatgaaatcttgaagatccatgaaaaaaacagtttattagaacataaaatcttagaaatggaaggaaaacacaaggaagagttggacaccttaaaggaagagaaagagaaccttcaaggcttggttactcgtcaaacatatataatccaggagctggaaaagcaattaaacagagctaccaccaacaacagtgtccttcagaagcagcaactggagctgatggacacagtccacaaccttgtcaatctttgcactaaagaaggtgttttactaaagggaggaaaaagagaggaagagaaaccatttagagactgtgcagatgtatatcaagctggttttaataaaagtggaatctacactatttatattaataatatgccagaacccaaaaaggtgttttgcaatatggatgtcaatgggggaggttggactgtaatacaacatcgtgaagatggaagtctagatttccaaagaggctggaaggaatataaaatgggttttggaaatccctccggtgaatattggctggggaatgagtttatttttgccattaccagtcagaggcagtacatgctaagaattgagttaatggactgggaagggaaccgagcctattcacagtatgacagattccacataggaaatgaaaagcaaaactataggttgtatttaaaaggtcacactgggacagcaggaaaacagagcagcctgatcttacacggtgctgatttcagcactaaagatgctgataatgacaactgtatgtgcaaatgtgccctcatgttaacaggaggatggtggtttgatgcttgtggcccctccaatctaaatggaatgttctatactgcgggacaaaaccatggaaaactgaatgggataaagtggcactacttcaaagggcccagttactccttacgttccacaactatgatgattcgacctttagatttttgaaagcgcaatgtcagaagcgattatgaaagcaacaaagaaatccggagaagctgccaggtgagaaactgtttgaaaacttcagaagcaaacaatattgtctcccttccagcaataagtggtagttatgtgaagtcaccaaggttcttgaccgtgaatctggagccgtttgagttcacaagagtctctacttggggtgacagtgctcacgtggctcgactatagaaaactccactgactgtcgggctttaaaaagggaagaaactgctgagcttgctgtgcttcaaactactactggaccttattttggaactatggtagccagatgataaatatggttaatttcatgtaaaacagaaaaaaagagtgaaaaagagaatatacatgaagaatagaaacaagcctgccataatcctttggaaaagatgtattataccagtgaaaaggtgttatatctatgcaaacctactaacaaattatactgttgcacaattttgataaaaatttagaacagcattgtcctctgagttggttaaatgttaatggatttcagaagcctaattccagtatcatacttactagttgatttctgcttacccatcttcaaatgaaaattccatttttgtaagccataatgaactgtagtacatggacaataagtgtgtggtagaaacaaactccattactctgatttttgatacagttttcagaaaaagaaatgaacataatcaagtaaggatgtatgtggtgaaaacttaccacccccatactatggttttcatttactctaaaaactgattgaatgatatataaatatatttatagcctgagtaaagttaaaagaatgtaaaatatatcatcaagttcttaaaataatatacatgcatttaatatttcctttgatattatacaggaaagcaatattttggagtatgttaagttgaagtaaaagcaagtactctggagcagttcattttacagtatctacttgcatgtgtatacatacatgtaacttcattattttaaaaatatttttagaactccaatactcaccctgttatgtcttgctaatttaaattttgctaattaactgaaacatgcttaccagattcacactgttccagtgtctataaaagaaacactttgaagtctataaaaaataaaataattataaatatcattgtacatagcatgtttatatctgcaaaaaacctaatagctaattaatctggaatatgcaacattgtccttaattgatgcaaataacacaaatgctcaaagaaatctactatatcccttaatgaaatacatcattcttcatatatttctccttcagtccattcccttaggcaatttttaatttttaaaaattattatcaggggagaaaaattggcaaaactattatatgtaagggaaatatatacaaaaagaaaattaatcatagtcacctgactaagaaattctgactgctagttgccataaataactcaatggaaatattcctatgggataatgtattttaagtgaatttttggggtgcttgaagttactgcattattttatcaagaagtcttctctgcctgtaagtgtccaaggttatgacagtaaacagtttttattaaaacatgagtcactatgggatgagaaaattgaaataaagctactgggcctcctctcataaaagagacagttgttggcaaggtagcaataccagtttcaaacttggtgacttgatccactatgccttaatggtttcctccatttgagaaaataaagctattcacattgttaagaaaaatactttttaaagtttaccatcaagtcttttttatatttatgtgtctgtattctacccctttttgccttacaagtgatatttgcaggtattataccatttttctattcttggtggcttcttcatagcaggtaagcctctccttctaaaaacttctcaactgttttcatttaagggaaagaaaatgagtattttgtccttttgtgttcctacagacactttcttaaaccagtttttggataaagaatactatttccaaactcatattacaaaaacaaaataaaataataaaaaaagaaagcatgatatttactgttttgttgtctgggtttgagaaatgaaatattgtttccaattatttataataaatcagtataaaatgttttatgattgttatgtgtattatgtaatacgtacatgtttatggcaatttaacatgtgtattcttttaattgtttcagaataggataattaggtattcgaattttgtctttaaaattcatgtggtttctatgcaaagttcttcatatcatcacaacattatttgatttaaataaaattgaaagtaatatttgtgcaa

SEQ ID NO: 49 - DNA, 3782 bp, Artificial Sequence
  Synthetic
gccctaagccatcagcaatccttagtataggggcacactcatgcattcctgtcaagtcatcttgtgaaaggctgcctgcttccagcttggcttggatgtgcaaccttaataaaactcactgaggtctgggagaaaatagcagatctgcagcagatagggtagaggaaagggtctagaatatgtacacgcagctgactcaggcaggctccatgctgaacggtcacacagagaggaaacaataaatctcagctactatgcaataaatatctcaagttttaacgaagaaaaacatcattgcagtgaaataaaaaattttaaaattttagaacaaagctaacaaatggctagttttctatgattcttcttcaaacgctttctttgagggggaaagagtcaaacaaacaagcagttttacctgaaataaagaactagttttagaggtcagaagaaaggagcaagttttgcgagaggcacggaaggagtgtgctggcagtacaatgacagttttcctttcctttgctttcctcgctgccattctgactgggatcttagacctagccccacagatgcttcgagaactccaggagactaatgcggcgctgcaagacgtgagagagctcttgcgacagcaggtcaaggagatcaccttcctgaagaatacggtgatggaatgtgacgcttgcggaggctcccttgtcaatctttgcactaaagaaggtgttttactaaagggaggaaaaagagaggaagagaaaccatttagagactgtgcagatgtatatcaagctggttttaataaaagtggaatctacactatttatattaataatatgccagaacccaaaaaggtgttttgcaatatggatgtcaatgggggaggttggactgtaatacaacatcgtgaagatggaagtctagatttccaaagaggctggaaggaatataaaatgggttttggaaatccctccggtgaatattggctggggaatgagtttatttttgccattaccagtcagaggcagtacatgctaagaattgagttaatggactgggaagggaaccgagcctattcacagtatgacagattccacataggaaatgaaaagcaaaactataggttgtatttaaaaggtcacactgggacagcaggaaaacagagcagcctgatcttacacggtgctgatttcagcactaaagatgctgataatgacaactgtatgtgcaaatgtgccctcatgttaacaggaggatggtggtttgatgcttgtggcccctccaatctaaatggaatgttctatactgcgggacaaaaccatggaaaactgaatgggataaagtggcactacttcaaagggcccagttactccttacgttccacaactatgatgattcgacctttagatttttgaaagcgcaatgtcagaagcgattatgaaagcaacaaagaaatccggagaagctgccaggtgagaaactgtttgaaaacttcagaagcaaacaatattgtctcccttccagcaataagtggtagttatgtgaagtcaccaaggttcttgaccgtgaatctggagccgtttgagttcacaagagtctctacttggggtgacagtgctcacgtggctcgactatagaaaactccactgactgtcgggctttaaaaagggaagaaactgctgagcttgctgtgcttcaaactactactggaccttattttggaactatggtagccagatgataaatatggttaatttcatgtaaaacagaaaaaaagagtgaaaaagagaatatacatgaagaatagaaacaagcctgccataatcctttggaaaagatgtattataccagtgaaaaggtgttatatctatgcaaacctactaacaaattatactgttgcacaattttgataaaaatttagaacagcattgtcctctgagttggttaaatgttaatggatttcagaagcctaattccagtatcatacttactagttgatttctgcttacccatcttcaaatgaaaattccatttttgtaagccataatgaactgtagtacatggacaataagtgtgtggtagaaacaaactccattactctgatttttgatacagttttcagaaaaagaaatgaacataatcaagtaaggatgtatgtggtgaaaacttaccacccccatactatggttttcatttactctaaaaactgattgaatgatatataaatatatttatagcctgagtaaagttaaaagaatgtaaaatatatcatcaagttcttaaaataatatacatgcatttaatatttcctttgatattatacaggaaagcaatattttggagtatgttaagttgaagtaaaagcaagtactctggagcagttcattttacagtatctacttgcatgtgtatacatacatgtaacttcattattttaaaaatatttttagaactccaatactcaccctgttatgtcttgctaatttaaattttgctaattaactgaaacatgcttaccagattcacactgttccagtgtctataaaagaaacactttgaagtctataaaaaataaaataattataaatatcattgtacatagcatgtttatatctgcaaaaaacctaatagctaattaatctggaatatgcaacattgtccttaattgatgcaaataacacaaatgctcaaagaaatctactatatcccttaatgaaatacatcattcttcatatatttctccttcagtccattcccttaggcaatttttaatttttaaaaattattatcaggggagaaaaattggcaaaactattatatgtaagggaaatatatacaaaaagaaaattaatcatagtcacctgactaagaaattctgactgctagttgccataaataactcaatggaaatattcctatgggataatgtattttaagtgaatttttggggtgcttgaagttactgcattattttatcaagaagtcttctctgcctgtaagtgtccaaggttatgacagtaaacagtttttattaaaacatgagtcactatgggatgagaaaattgaaataaagctactgggcctcctctcataaaagagacagttgttggcaaggtagcaataccagtttcaaacttggtgacttgatccactatgccttaatggtttcctccatttgagaaaataaagctattcacattgttaagaaaaatactttttaaagtttaccatcaagtcttttttatatttatgtgtctgtattctacccctttttgccttacaagtgatatttgcaggtattataccatttttctattcttggtggcttcttcatagcaggtaagcctctccttctaaaaacttctcaactgttttcatttaagggaaagaaaatgagtattttgtccttttgtgttcctacagacactttcttaaaccagtttttggataaagaatactatttccaaactcatattacaaaaacaaaataaaataataaaaaaagaaagcatgatatttactgttttgttgtctgggtttgagaaatgaaatattgtttccaattatttataataaatcagtataaaatgttttatgattgttatgtgtattatgtaatacgtacatgtttatggcaatttaacatgtgtattcttttaattgtttcagaataggataattaggtattcgaattttgtctttaaaattcatgtggtttctatgcaaagttcttcatatcatcacaacattatttgatttaaataaaattgaaagtaatatttgtgcaa

SEQ ID NO: 50 - DNA, 1976 bp, Artificial Sequence
  Synthetic
aaagtgattgattcggatactgacactgtaggatctggggagagaggaacaaaggaccgtgaaagctgctctgtaaaagctgacacagccctcccaagtgagcaggactgttcttcccactgcaatctgacagtttactgcatgcctggagagaacacagcagtaaaaaccaggtttgctactggaaaaagaggaaagagaagactttcattgacggacccagccatggcagcgtagcagccctgcgttttagacggcagcagctcgggactctggacgtgtgtttgccctcaagtttgctaagctgctggtttattactgaagaaagaatgtggcagattgttttctttactctgagctgtgatcttgtcttggccgcagcccacatagggtgcagcaatcagcgccgaagtccagaaaacagtgggagaagatataaccggattcaacatgggcaatgtgcctacactttcattcttccagaacacgatggcaactgtcgtgagagtacgacagaccagtacaacacaaacgctctgcagagagatgctccacacgtggaaccggatttctcttcccagaaacttcaacatctggaacatgtgatggaaaattatactcagtggctgcaaaaacttgagaattacattgtggaaaacatgaagtcggagatggcccagatacagcagaatgcagttcagaaccacacggctaccatgctggagataggaaccagcctcctctctcagactgcagagcagaccagaaagctgacagatgttgagacccaggtactaaatcaaacttctcgacttgagatacagctgctggagaattcattatccacctacaagctagagaagcaacttcttcaacagacaaatgaaatcttgaagatccatgaaaaaaacagtttattagaacataaaatcttagaaatggaaggaaaacacaaggaagagttggacaccttaaaggaagagaaagagaaccttcaaggcttggttactcgtcaaacatatataatccaggagctggaaaagcaattaaacagagctaccaccaacaacagtgtccttcagaagcagcaactggagctgatggacacagtccacaaccttgtcaatctttgcactaaagaaggtgttttactaaagggaggaaaaagagaggaagagaaaccatttagagactgtgcagatgtatatcaagctggttttaataaaagtggaatctacactatttatattaataatatgccagaacccaaaaaggtgttttgcaatatggatgtcaatgggggaggttggactgtaatacaacatcgtgaagatggaagtctagatttccaaagaggctggaaggaatataaaatgggttttggaaatccctccggtgaatattggctggggaatgagtttatttttgccattaccagtcagaggcagtacatgctaagaattgagttaatggactgggaagggaaccgagcctattcacagtatgacagattccacataggaaatgaaaagcaaaactataggttgtatttaaaaggtcacactgggacagcaggaaaacagagcagcctgatcttacacggtgctgatttcagcactaaagatgctgataatgacaactgtatgtgcaaatgtgccctcatgttaacaggaggatggtggtttgatgcttgtggcccctccaatctaaatggaatgttctatactgcgggacaaaaccatggaaaactgaatgggataaagtggcactacttcaaagggcccagttactccttacgttccacaactatgatgattcgacctttagatttttgaggctgctgcagctgcatgggtgcctgctgctgcctgccttggcctgatggccaggccagagtgctgccagtcctctgcatgttctgctcttgtgcccttctgagcccacaataaaggctgagctcttatcttgcaaaaggc

SEQ ID NO: 51 - DNA, 1391 bp, Artificial Sequence
  Synthetic
aaagtgattgattcggatactgacactgtaggatctggggagagaggaacaaaggaccgtgaaagctgctctgtaaaagctgacacagccctcccaagtgagcaggactgttcttcccactgcaatctgacagtttactgcatgcctggagagaacacagcagtaaaaaccaggtttgctactggaaaaagaggaaagagaagactttcattgacggacccagccatggcagcgtagcagccctgcgttttagacggcagcagctcgggactctggacgtgtgtttgccctcaagtttgctaagctgctggtttattactgaagaaagaatgtggcagattgttttctttactctgagctgtgatcttgtcttggccgcagccgggatcttagacctagccccacagatgcttcgagaactccaggagactaatgcggcgctgcaagacgtgagagagctcttgcgacagcaggtcaaggagatcaccttcctgaagaatacggtgatggaatgtgacgcttgcggaggctcccttgtcaatctttgcactaaagaaggtgttttactaaagggaggaaaaagagaggaagagaaaccatttagagactgtgcagatgtatatcaagctggttttaataaaagtggaatctacactatttatattaataatatgccagaacccaaaaaggtgttttgcaatatggatgtcaatgggggaggttggactgtaatacaacatcgtgaagatggaagtctagatttccaaagaggctggaaggaatataaaatgggttttggaaatccctccggtgaatattggctggggaatgagtttatttttgccattaccagtcagaggcagtacatgctaagaattgagttaatggactgggaagggaaccgagcctattcacagtatgacagattccacataggaaatgaaaagcaaaactataggttgtatttaaaaggtcacactgggacagcaggaaaacagagcagcctgatcttacacggtgctgatttcagcactaaagatgctgataatgacaactgtatgtgcaaatgtgccctcatgttaacaggaggatggtggtttgatgcttgtggcccctccaatctaaatggaatgttctatactgcgggacaaaaccatggaaaactgaatgggataaagtggcactacttcaaagggcccagttactccttacgttccacaactatgatgattcgacctttagatttttgaggctgctgcagctgcatgggtgcctgctgctgcctgccttggcctgatggccaggccagagtgctgccagtcctctgcatgttctgctcttgtgcccttctgagcccacaataaaggctgagctcttatcttgcaaaaggc

SEQ ID NO: 52 - DNA, 1967 bp, Artificial Sequence
  Synthetic
gaggaaccgagaggctgagactaacccagaaacatccaattctcaaactgaagctcgcactctcgcctccagcatgaaagtctctgccgcccttctgtgcctgctgctcatagcagccaccttcattccccaagggctcgctcacatagggtgcagcaatcagcgccgaagtccagaaaacagtgggagaagatataaccggattcaacatgggcaatgtgcctacactttcattcttccagaacacgatggcaactgtcgtgagagtacgacagaccagtacaacacaaacgctctgcagagagatgctccacacgtggaaccggatttctcttcccagaaacttcaacatctggaacatgtgatggaaaattatactcagtggctgcaaaaacttgagaattacattgtggaaaacatgaagtcggagatggcccagatacagcagaatgcagttcagaaccacacggctaccatgctggagataggaaccagcctcctctctcagactgcagagcagaccagaaagctgacagatgttgagacccaggtactaaatcaaacttctcgacttgagatacagctgctggagaattcattatccacctacaagctagagaagcaacttcttcaacagacaaatgaaatcttgaagatccatgaaaaaaacagtttattagaacataaaatcttagaaatggaaggaaaacacaaggaagagttggacaccttaaaggaagagaaagagaaccttcaaggcttggttactcgtcaaacatatataatccaggagctggaaaagcaattaaacagagctaccaccaacaacagtgtccttcagaagcagcaactggagctgatggacacagtccacaaccttgtcaatctttgcactaaagaaggtgttttactaaagggaggaaaaagagaggaagagaaaccatttagagactgtgcagatgtatatcaagctggttttaataaaagtggaatctacactatttatattaataatatgccagaacccaaaaaggtgttttgcaatatggatgtcaatgggggaggttggactgtaatacaacatcgtgaagatggaagtctagatttccaaagaggctggaaggaatataaaatgggttttggaaatccctccggtgaatattggctggggaatgagtttatttttgccattaccagtcagaggcagtacatgctaagaattgagttaatggactgggaagggaaccgagcctattcacagtatgacagattccacataggaaatgaaaagcaaaactataggttgtatttaaaaggtcacactgggacagcaggaaaacagagcagcctgatcttacacggtgctgatttcagcactaaagatgctgataatgacaactgtatgtgcaaatgtgccctcatgttaacaggaggatggtggtttgatgcttgtggcccctccaatctaaatggaatgttctatactgcgggacaaaaccatggaaaactgaatgggataaagtggcactacttcaaagggcccagttactccttacgttccacaactatgatgattcgacctttagatttttgaacactcactccacaacccaagaatctgcagctaacttattttcccctagctttccccagacaccctgttttattttattataatgaattttgtttgttgatgtgaaacattatgccttaagtaatgttaattcttatttaagttattgatgttttaagtttatctttcatggtactagtgttttttagatacagagacttggggaaattgcttttcctcttgaaccacagttctacccctgggatgttttgagggtctttgcaagaatcattaatacaaagaattttttttaacattccaatgcattgctaaaatattattgtggaaatgaatattttgtaactattacaccaaataaatatatttttgtaca

SEQ ID NO: 53 - DNA, 1382 bp, Artificial Sequence
  Synthetic
gaggaaccgagaggctgagactaacccagaaacatccaattctcaaactgaagctcgcactctcgcctccagcatgaaagtctctgccgcccttctgtgcctgctgctcatagcagccaccttcattccccaagggctcgctgggatcttagacttgggcccgcagatgcttcgggaactgcaggaaaccaacgcggcgctgcaggacgtgcgggagctgctgcggcagcaggtcagggagatcacgttcctgaaaaacacggtgatggagtgtgacgcgtgcggaggctcccttgtcaatctttgcactaaagaaggtgttttactaaagggaggaaaaagagaggaagagaaaccatttagagactgtgcagatgtatatcaagctggttttaataaaagtggaatctacactatttatattaataatatgccagaacccaaaaaggtgttttgcaatatggatgtcaatgggggaggttggactgtaatacaacatcgtgaagatggaagtctagatttccaaagaggctggaaggaatataaaatgggttttggaaatccctccggtgaatattggctggggaatgagtttatttttgccattaccagtcagaggcagtacatgctaagaattgagttaatggactgggaagggaaccgagcctattcacagtatgacagattccacataggaaatgaaaagcaaaactataggttgtatttaaaaggtcacactgggacagcaggaaaacagagcagcctgatcttacacggtgctgatttcagcactaaagatgctgataatgacaactgtatgtgcaaatgtgccctcatgttaacaggaggatggtggtttgatgcttgtggcccctccaatctaaatggaatgttctatactgcgggacaaaaccatggaaaactgaatgggataaagtggcactacttcaaagggcccagttactccttacgttccacaactatgatgattcgacctttagatttttgaacactcactccacaacccaagaatctgcagctaacttattttcccctagctttccccagacaccctgttttattttattataatgaattttgtttgttgatgtgaaacattatgccttaagtaatgttaattcttatttaagttattgatgttttaagtttatctttcatggtactagtgttttttagatacagagacttggggaaattgcttttcctcttgaaccacagttctacccctgggatgttttgagggtctttgcaagaatcattaatacaaagaattttttttaacattccaatgcattgctaaaatattattgtggaaatgaatattttgtaactattacaccaaataaatatatttttgtaca

SEQ ID NO: 54 - DNA, 3428 bp, Artificial Sequence
  Synthetic
gccctaagccatcagcaatccttagtataggggcacactcatgcattcctgtcaagtcatcttgtgaaaggctgcctgcttccagcttggcttggatgtgcaaccttaataaaactcactgaggtctgggagaaaatagcagatctgcagcagatagggtagaggaaagggtctagaatatgtacacgcagctgactcaggcaggctccatgctgaacggtcacacagagaggaaacaataaatctcagctactatgcaataaatatctcaagttttaacgaagaaaaacatcattgcagtgaaataaaaaattttaaaattttagaacaaagctaacaaatggctagttttctatgattcttcttcaaacgctttctttgagggggaaagagtcaaacaaacaagcagttttacctgaaataaagaactagttttagaggtcagaagaaaggagcaagttttgcgagaggcacggaaggagtgtgctggcagtacaatgacagttttcctttcctttgctttcctcgctgccattctgactgtcttcacactcgaagatttcgttggggactggcgacagacagccggctacaacctggaccaagtccttgaacagggaggtgtgtccagtttgtttcagaatctcggggtgtccgtaactccgatccaaaggattgtcctgagcggtgaaaatgggctgaagatcgacatccatgtcatcatcccgtatgaaggtctgagcggcgaccaaatgggccagatcgaaaaaatttttaaggtggtgtaccctgtggatgatcatcactttaaggtgatcctgcactatggcacactggtaatcgacggggttacgccgaacatgatcgactatttcggacggccgtatgaaggcatcgccgtgttcgacggcaaaaagatcactgtaacagggaccctgtggaacggcaacaaaattatcgacgagcgcctgatcaaccccgacggctccctgctgttccgagtaaccatcaacggagtgaccggctggcggctgtgcgaacgcattctggcgtaaaagcgcaatgtcagaagcgattatgaaagcaacaaagaaatccggagaagctgccaggtgagaaactgtttgaaaacttcagaagcaaacaatattgtctcccttccagcaataagtggtagttatgtgaagtcaccaaggttcttgaccgtgaatctggagccgtttgagttcacaagagtctctacttggggtgacagtgctcacgtggctcgactatagaaaactccactgactgtcgggctttaaaaagggaagaaactgctgagcttgctgtgcttcaaactactactggaccttattttggaactatggtagccagatgataaatatggttaatttcatgtaaaacagaaaaaaagagtgaaaaagagaatatacatgaagaatagaaacaagcctgccataatcctttggaaaagatgtattataccagtgaaaaggtgttatatctatgcaaacctactaacaaattatactgttgcacaattttgataaaaatttagaacagcattgtcctctgagttggttaaatgttaatggatttcagaagcctaattccagtatcatacttactagttgatttctgcttacccatcttcaaatgaaaattccatttttgtaagccataatgaactgtagtacatggacaataagtgtgtggtagaaacaaactccattactctgatttttgatacagttttcagaaaaagaaatgaacataatcaagtaaggatgtatgtggtgaaaacttaccacccccatactatggttttcatttactctaaaaactgattgaatgatatataaatatatttatagcctgagtaaagttaaaagaatgtaaaatatatcatcaagttcttaaaataatatacatgcatttaatatttcctttgatattatacaggaaagcaatattttggagtatgttaagttgaagtaaaagcaagtactctggagcagttcattttacagtatctacttgcatgtgtatacatacatgtaacttcattattttaaaaatatttttagaactccaatactcaccctgttatgtcttgctaatttaaattttgctaattaactgaaacatgcttaccagattcacactgttccagtgtctataaaagaaacactttgaagtctataaaaaataaaataattataaatatcattgtacatagcatgtttatatctgcaaaaaacctaatagctaattaatctggaatatgcaacattgtccttaattgatgcaaataacacaaatgctcaaagaaatctactatatcccttaatgaaatacatcattcttcatatatttctccttcagtccattcccttaggcaatttttaatttttaaaaattattatcaggggagaaaaattggcaaaactattatatgtaagggaaatatatacaaaaagaaaattaatcatagtcacctgactaagaaattctgactgctagttgccataaataactcaatggaaatattcctatgggataatgtattttaagtgaatttttggggtgcttgaagttactgcattattttatcaagaagtcttctctgcctgtaagtgtccaaggttatgacagtaaacagtttttattaaaacatgagtcactatgggatgagaaaattgaaataaagctactgggcctcctctcataaaagagacagttgttggcaaggtagcaataccagtttcaaacttggtgacttgatccactatgccttaatggtttcctccatttgagaaaataaagctattcacattgttaagaaaaatactttttaaagtttaccatcaagtcttttttatatttatgtgtctgtattctacccctttttgccttacaagtgatatttgcaggtattataccatttttctattcttggtggcttcttcatagcaggtaagcctctccttctaaaaacttctcaactgttttcatttaagggaaagaaaatgagtattttgtccttttgtgttcctacagacactttcttaaaccagtttttggataaagaatactatttccaaactcatattacaaaaacaaaataaaataataaaaaaagaaagcatgatatttactgttttgttgtctgggtttgagaaatgaaatattgtttccaattatttataataaatcagtataaaatgttttatgattgttatgtgtattatgtaatacgtacatgtttatggcaatttaacatgtgtattcttttaattgtttcagaataggataattaggtattcgaattttgtctttaaaattcatgtggtttctatgcaaagttcttcatatcatcacaacattatttgatttaaataaaattgaaagtaatatttgtgcaa

SEQ ID NO: 55 - DNA, 1037 bp, Artificial Sequence
  Synthetic
aaagtgattgattcggatactgacactgtaggatctggggagagaggaacaaaggaccgtgaaagctgctctgtaaaagctgacacagccctcccaagtgagcaggactgttcttcccactgcaatctgacagtttactgcatgcctggagagaacacagcagtaaaaaccaggtttgctactggaaaaagaggaaagagaagactttcattgacggacccagccatggcagcgtagcagccctgcgttttagacggcagcagctcgggactctggacgtgtgtttgccctcaagtttgctaagctgctggtttattactgaagaaagaatgtggcagattgttttctttactctgagctgtgatcttgtcttggccgcagccgtcttcacactcgaagatttcgttggggactggcgacagacagccggctacaacctggaccaagtccttgaacagggaggtgtgtccagtttgtttcagaatctcggggtgtccgtaactccgatccaaaggattgtcctgagcggtgaaaatgggctgaagatcgacatccatgtcatcatcccgtatgaaggtctgagcggcgaccaaatgggccagatcgaaaaaatttttaaggtggtgtaccctgtggatgatcatcactttaaggtgatcctgcactatggcacactggtaatcgacggggttacgccgaacatgatcgactatttcggacggccgtatgaaggcatcgccgtgttcgacggcaaaaagatcactgtaacagggaccctgtggaacggcaacaaaattatcgacgagcgcctgatcaaccccgacggctccctgctgttccgagtaaccatcaacggagtgaccggctggcggctgtgcgaacgcattctggcgtaaggctgctgcagctgcatgggtgcctgctgctgcctgccttggcctgatggccaggccagagtgctgccagtcctctgcatgttctgctcttgtgcccttctgagcccacaataaaggctgagctcttatcttgcaaaaggc

SEQ ID NO: 56 - DNA, 826 bp, Artificial Sequence
  Synthetic
tccccattgaataacagccaagttgctttggtttctatttctttgttaagtcgttccctctacaaaggacttcctagtgggtgtgaaaggcagcggtggccacagaggcggcggagagatgtggcagattgttttctttactctgagctgtgatcttgtcttggccgcagccgtcttcacactcgaagatttcgttggggactggcgacagacagccggctacaacctggaccaagtccttgaacagggaggtgtgtccagtttgtttcagaatctcggggtgtccgtaactccgatccaaaggattgtcctgagcggtgaaaatgggctgaagatcgacatccatgtcatcatcccgtatgaaggtctgagcggcgaccaaatgggccagatcgaaaaaatttttaaggtggtgtaccctgtggatgatcatcactttaaggtgatcctgcactatggcacactggtaatcgacggggttacgccgaacatgatcgactatttcggacggccgtatgaaggcatcgccgtgttcgacggcaaaaagatcactgtaacagggaccctgtggaacggcaacaaaattatcgacgagcgcctgatcaaccccgacggctccctgctgttccgagtaaccatcaacggagtgaccggctggcggctgtgcgaacgcattctggcgtaaggctgctgcagctgcatgggtgcctgctgctgcctgccttggcctgatggccaggccagagtgctgccagtcctctgcatgttctgctcttgtgcccttctgagcccacaataaaggctgagctcttatcttgcaaaaggc

SEQ ID NO: 57 - DNA, 1068 bp, Artificial Sequence
  Synthetic
ataaaagcccaggggcaagcggtccggataacggctagcctgaggagctgctgcgacagtccactacctttttcgagagtgactcccgttgtcccaaggcttcccagagcgaacctgtgcggctgcaggcaccggcgcgtcgagtttccggcgtccggaaggaccgagctcttctcgcgaatccagtgttccgtttccagcccccaatctcagagcggagccgacagagagcagggaaccggcatgtggcagattgttttctttactctgagctgtgatcttgtcttggccgcagccgtcttcacactcgaagatttcgttggggactggcgacagacagccggctacaacctggaccaagtccttgaacagggaggtgtgtccagtttgtttcagaatctcggggtgtccgtaactccgatccaaaggattgtcctgagcggtgaaaatgggctgaagatcgacatccatgtcatcatcccgtatgaaggtctgagcggcgaccaaatgggccagatcgaaaaaatttttaaggtggtgtaccctgtggatgatcatcactttaaggtgatcctgcactatggcacactggtaatcgacggggttacgccgaacatgatcgactatttcggacggccgtatgaaggcatcgccgtgttcgacggcaaaaagatcactgtaacagggaccctgtggaacggcaacaaaattatcgacgagcgcctgatcaaccccgacggctccctgctgttccgagtaaccatcaacggagtgaccggctggcggctgtgcgaacgcattctggcgtaagggcctttccaagattgctgtttttgttttggagcttcaagactttgcatttcctagtatttctgtttgtcagttctcaatttcctgtgtttgcaatgttgaaattttttggtgaagtactgaacttgctttttttccggtttctacatgcagagatgaatttatactgccatcttacgactatttcttctttttaatacacttaactcaggccattttttaagttggttacttcaaagtaaataaactttaaaattc

SEQ ID NO: 58 - DNA, 1217 bp, Artificial Sequence
  Synthetic
gtcagccatctttcaattgtgttcgcagccgccgccgcgccgccgtcgctctccaacgccagcgccgcctctcgctcgccgagctccagccgaaggagaaggggggtaagtaaggaggtctctgtaccatgtggcagattgttttctttactctgagctgtgatcttgtcttggccgcagccgtcttcacactcgaagatttcgttggggactggcgacagacagccggctacaacctggaccaagtccttgaacagggaggtgtgtccagtttgtttcagaatctcggggtgtccgtaactccgatccaaaggattgtcctgagcggtgaaaatgggctgaagatcgacatccatgtcatcatcccgtatgaaggtctgagcggcgaccaaatgggccagatcgaaaaaatttttaaggtggtgtaccctgtggatgatcatcactttaaggtgatcctgcactatggcacactggtaatcgacggggttacgccgaacatgatcgactatttcggacggccgtatgaaggcatcgccgtgttcgacggcaaaaagatcactgtaacagggaccctgtggaacggcaacaaaattatcgacgagcgcctgatcaaccccgacggctccctgctgttccgagtaaccatcaacggagtgaccggctggcggctgtgcgaacgcattctggcgtaagaatccactatgatgggaaacatttcattctcaaaaaaaaaaaaaaaaatttctcttcttcctgttattggtagttctgaacgttagatattttttttccatggggtcaaaaggtacctaagtatatgattgcgagtggaaaaataggggacagaaatcaggtattggcagtttttccattttcatttgtgtgtgaatttttaatataaatgcggagacgtaaagcattaatgcaagttaaaatgtttcagtgaacaagtttcagcggttcaactttataataattataaataaacctgttaaatttttctggacaatgccagcatttggatttttttaaaacaagtaaatttcttattgatggcaactaaatggtgtttgtagcatttttatcatacagtagattccatccattcactatacttttctaactgagttgtcctacatgcaagtacatgtttttaatgttgtctgtcttctgtgctgttcctgtaagtttgctattaaaatacattaaactat

SEQ ID NO: 59 - DNA, 827 bp, Artificial Sequence
  Synthetic
catatcttcattcttcactctttccccccccccccttatcctcctatctaatcctctcatctctctcctcctcttcctccaacaacaactaacaatggcagcaactacaacaatggcacagattgttttctttactctgagctgtgatcttgtcttggccgcagccgtcttcacactcgaagatttcgttggggactggcgacagacagccggctacaacctggaccaagtccttgaacagggaggtgtgtccagtttgtttcagaatctcggggtgtccgtaactccgatccaaaggattgtcctgagcggtgaaaatgggctgaagatcgacatccatgtcatcatcccgtatgaaggtctgagcggcgaccaaatgggccagatcgaaaaaatttttaaggtggtgtaccctgtggatgatcatcactttaaggtgatcctgcactatggcacactggtaatcgacggggttacgccgaacatgatcgactatttcggacggccgtatgaaggcatcgccgtgttcgacggcaaaaagatcactgtaacagggaccctgtggaacggcaacaaaattatcgacgagcgcctgatcaaccccgacggctccctgctgttccgagtaaccatcaacggagtgaccggctggcggctgtgcgaacgcattctggcgtaattttgagtaattttcaattttgtttttgtttttgtttttgttgttgggagttgttgtaatttggtaaatgttggggtcactaaaatcttttgttgcaattttagcacctttttattagatatataaaattgggtttagatgtagttaa

SEQ ID NO: 60 - DNA, 925 bp, Artificial Sequence
  Synthetic
ataaaagcctagtggccattgtgttcgttgctcttatcggttcccatcccagttgttgatcttatgcaagacgctgcacgaccccgcgcccgcttgtcgccacggcacttgaggcagccggagatactctgagttactcggagcccgacgcctgagggtgagatgaacgcgctggcctccctaaccgtccggacctgtgatcgcttctggcagaccgaaccggcgctcctgcccccggggtgacgcgcagctcccagccgcccagacacatgtggcagattgttttctttactctgagctgtgatcttgtcttggccgcagccgtcttcacactcgaagatttcgttggggactggcgacagacagccggctacaacctggaccaagtccttgaacagggaggtgtgtccagtttgtttcagaatctcggggtgtccgtaactccgatccaaaggattgtcctgagcggtgaaaatgggctgaagatcgacatccatgtcatcatcccgtatgaaggtctgagcggcgaccaaatgggccagatcgaaaaaatttttaaggtggtgtaccctgtggatgatcatcactttaaggtgatcctgcactatggcacactggtaatcgacggggttacgccgaacatgatcgactatttcggacggccgtatgaaggcatcgccgtgttcgacggcaaaaagatcactgtaacagggaccctgtggaacggcaacaaaattatcgacgagcgcctgatcaaccccgacggctccctgctgttccgagtaaccatcaacggagtgaccggctggcggctgtgcgaacgcattctggcgtaagaccaactggtttgcctataatttattaactatttattttttctaagtgtgggtttatataaggaataaagccttttgatttgtagcga

SEQ ID NO: 61 - DNA, 1028 bp, Artificial Sequence
  Synthetic
gaggaaccgagaggctgagactaacccagaaacatccaattctcaaactgaagctcgcactctcgcctccagcatgaaagtctctgccgcccttctgtgcctgctgctcatagcagccaccttcattccccaagggctcgctgtcttcacactcgaagatttcgttggggactggcgacagacagccggctacaacctggaccaagtccttgaacagggaggtgtgtccagtttgtttcagaatctcggggtgtccgtaactccgatccaaaggattgtcctgagcggtgaaaatgggctgaagatcgacatccatgtcatcatcccgtatgaaggtctgagcggcgaccaaatgggccagatcgaaaaaatttttaaggtggtgtaccctgtggatgatcatcactttaaggtgatcctgcactatggcacactggtaatcgacggggttacgccgaacatgatcgactatttcggacggccgtatgaaggcatcgccgtgttcgacggcaaaaagatcactgtaacagggaccctgtggaacggcaacaaaattatcgacgagcgcctgatcaaccccgacggctccctgctgttccgagtaaccatcaacggagtgaccggctggcggctgtgcgaacgcattctggcgtaaacactcactccacaacccaagaatctgcagctaacttattttcccctagctttccccagacaccctgttttattttattataatgaattttgtttgttgatgtgaaacattatgccttaagtaatgttaattcttatttaagttattgatgttttaagtttatctttcatggtactagtgttttttagatacagagacttggggaaattgcttttcctcttgaaccacagttctacccctgggatgttttgagggtctttgcaagaatcattaatacaaagaattttttttaacattccaatgcattgctaaaatattattgtggaaatgaatattttgtaactattacaccaaataaatatatttttgtaca

SEQ ID NO: 62 - DNA, 2027 bp, Artificial Sequence
  Synthetic
ggagctgtttacccccactctaataggggttcaatataaaaagccggcagagagctgtccaagtcagacgcgcctctgcatctgcgccaggcgaacgggtcctgcgcctcctgcagtcccagctctccaccgccgcgtgcgcctgcagacgctccgctcgctgccttctctcctggcaggcgctgccttttctccccgttaaaagggcacttgggctgaaggatcgctttgagatctgaggaacccgcagcgctttgagggacctgaagctgtttttcttcgttttcctttgggttcagtttgaacgggaggtttttgatccctttttttcagaatggattatttgctcatgattttctctctgctgtttgtggcttgccaaggagtcttcacactcgaagatttcgttggggactggcgacagacagccggctacaacctggaccaagtccttgaacagggaggtgtgtccagtttgtttcagaatctcggggtgtccgtaactccgatccaaaggattgtcctgagcggtgaaaatgggctgaagatcgacatccatgtcatcatcccgtatgaaggtctgagcggcgaccaaatgggccagatcgaaaaaatttttaaggtggtgtaccctgtggatgatcatcactttaaggtgatcctgcactatggcacactggtaatcgacggggttacgccgaacatgatcgactatttcggacggccgtatgaaggcatcgccgtgttcgacggcaaaaagatcactgtaacagggaccctgtggaacggcaacaaaattatcgacgagcgcctgatcaaccccgacggctccctgctgttccgagtaaccatcaacggagtgaccggctggcggctgtgcgaacgcattctggcgtaacagaccttcggggcctgtctgaagccatagcctccacggagagccctgtggccgactctgcactctccaccctggctgggatcagagcaggagcatcctctgctggttcctgactggcaaaggaccagcgtcctcgttcaaaacattccaagaaaggttaaggagttcccccaaccatcttcactggcttccatcagtggtaactgctttggtctcttctttcatctggggatgacaatggacctctcagcagaaacacacagtcacattcgaattcgggtggcatcctccggagagagagagaggaaggagattccacacaggggtggagtttctgacgaaggtcctaagggagtgtttgtgtctgactcaggcgcctggcacatttcagggagaaactccaaagtccacacaaagattttctaaggaatgcacaaattgaaaacacactcaaaagacaaacatgcaagtaaagaaaaaaaaaagaaagacttttgtttaaatttgtaaaatgcaaaactgaatgaaactgttactaccataaatcaggatatgtttcatgaatatgagtctacctcacctatattgcactctggcagaagtatttcccacatttaattattgcctccccaaactcttcccacccctgctgccccttcctccatcccccatactaaatcctagcctcgtagaagtctggtctaatgtgtcagcagtagatataatattttcatggtaatctactagctctgatccataagaaaaaaaagatcattaaatcaggagattccctgtccttgatttttggagacacaatggtatagggttgtttatgaaatatattgaaaagtaagtgtttgttacgctttaaagcagtaaaattattttcctttatataaccggctaatgaaagaggttggattgaattttgatgtacttatttttttatagatatttatattcaaacaatttattccttatatttaccatgttaaatatctgtttgggcaggccatattggtctatgtatttttaaaatatgtatttctaaatgaaattgagaacatgctttgttttgcctgtcaaggtaatgactttagaaaataaatatttttttccttactgtaaa

SEQ ID NO: 63 - DNA, 1070 bp, Artificial Sequence
  Synthetic
aaagtgattgattcggatactgacactgtaggatctggggagagaggaacaaaggaccgtgaaagctgctctgtaaaagctgacacagccctcccaagtgagcaggactgttcttcccactgcaatctgacagtttactgcatgcctggagagaacacagcagtaaaaaccaggtttgctactggaaaaagaggaaagagaagactttcattgacggacccagccatggcagcgtagcagccctgcgttttagacggcagcagctcgggactctggacgtgtgtttgccctcaagtttgctaagctgctggtttattactgaagaaagaatgaactccttctccacaagcgccttcggtccagttgccttctccctgggcctgctcctggtgttgcctgctgccttccctgccccagtcttcacactcgaagatttcgttggggactggcgacagacagccggctacaacctggaccaagtccttgaacagggaggtgtgtccagtttgtttcagaatctcggggtgtccgtaactccgatccaaaggattgtcctgagcggtgaaaatgggctgaagatcgacatccatgtcatcatcccgtatgaaggtctgagcggcgaccaaatgggccagatcgaaaaaatttttaaggtggtgtaccctgtggatgatcatcactttaaggtgatcctgcactatggcacactggtaatcgacggggttacgccgaacatgatcgactatttcggacggccgtatgaaggcatcgccgtgttcgacggcaaaaagatcactgtaacagggaccctgtggaacggcaacaaaattatcgacgagcgcctgatcaaccccgacggctccctgctgttccgagtaaccatcaacggagtgaccggctggcggctgtgcgaacgcattctggcgtaaggctgctgcagctgcatgggtgcctgctgctgcctgccttggcctgatggccaggccagagtgctgccagtcctctgcatgttctgctcttgtgcccttctgagcccacaataaaggctgagctcttatcttgcaaaaggc

SEQ ID NO: 64 - DNA, 796 bp, Artificial Sequence
  Synthetic
gaggaaccgagaggctgagactaacccagaaacatccaattctcaaactgaagctcgcactctcgcctccagcatgaaagtctctgccgcccttctgtgcctgctgctcatagcagccaccttcattccccaagggctcgctgtcttcacactcgaagatttcgttggggactggcgacagacagccggctacaacctggaccaagtccttgaacagggaggtgtgtccagtttgtttcagaatctcggggtgtccgtaactccgatccaaaggattgtcctgagcggtgaaaatgggctgaagatcgacatccatgtcatcatcccgtatgaaggtctgagcggcgaccaaatgggccagatcgaaaaaatttttaaggtggtgtaccctgtggatgatcatcactttaaggtgatcctgcactatggcacactggtaatcgacggggttacgccgaacatgatcgactatttcggacggccgtatgaaggcatcgccgtgttcgacggcaaaaagatcactgtaacagggaccctgtggaacggcaacaaaattatcgacgagcgcctgatcaaccccgacggctccctgctgttccgagtaaccatcaacggagtgaccggctggcggctgtgcgaacgcattctggcgtaaggctgctgcagctgcatgggtgcctgctgctgcctgccttggcctgatggccaggccagagtgctgccagtcctctgcatgttctgctcttgtgcccttctgagcccacaataaaggctgagctcttatcttgcaaaaggc

SEQ ID NO: 65 - DNA, 913 bp, Artificial Sequence
  Synthetic
gaggaaccgagaggctgagactaacccagaaacatccaattctcaaactgaagctcgcactctcgcctccagcatgaaagtctctgccgcccttctgtgcctgctgctcatagcagccaccttcattccccaagggctcgctgtcttcacactcgaagatttcgttggggactggcgacagacagccggctacaacctggaccaagtccttgaacagggaggtgtgtccagtttgtttcagaatctcggggtgtccgtaactccgatccaaaggattgtcctgagcggtgaaaatgggctgaagatcgacatccatgtcatcatcccgtatgaaggtctgagcggcgaccaaatgggccagatcgaaaaaatttttaaggtggtgtaccctgtggatgatcatcactttaaggtgatcctgcactatggcacactggtaatcgacggggttacgccgaacatgatcgactatttcggacggccgtatgaaggcatcgccgtgttcgacggcaaaaagatcactgtaacagggaccctgtggaacggcaacaaaattatcgacgagcgcctgatcaaccccgacggctccctgctgttccgagtaaccatcaacggagtgaccggctggcggctgtgcgaacgcattctggcgtaagggcctttccaagattgctgtttttgttttggagcttcaagactttgcatttcctagtatttctgtttgtcagttctcaatttcctgtgtttgcaatgttgaaattttttggtgaagtactgaacttgctttttttccggtttctacatgcagagatgaatttatactgccatcttacgactatttcttctttttaatacacttaactcaggccattttttaagttggttacttcaaagtaaataaactttaaaattc

SEQ ID NO: 66 - DNA, 1046 bp, Artificial Sequence
  Synthetic
gaggaaccgagaggctgagactaacccagaaacatccaattctcaaactgaagctcgcactctcgcctccagcatgaactccttctccacaagcgccttcggtccagttgccttctccctgggcctgctcctggtgttgcctgctgccttccctgccccagtcttcacactcgaagatttcgttggggactggcgacagacagccggctacaacctggaccaagtccttgaacagggaggtgtgtccagtttgtttcagaatctcggggtgtccgtaactccgatccaaaggattgtcctgagcggtgaaaatgggctgaagatcgacatccatgtcatcatcccgtatgaaggtctgagcggcgaccaaatgggccagatcgaaaaaatttttaaggtggtgtaccctgtggatgatcatcactttaaggtgatcctgcactatggcacactggtaatcgacggggttacgccgaacatgatcgactatttcggacggccgtatgaaggcatcgccgtgttcgacggcaaaaagatcactgtaacagggaccctgtggaacggcaacaaaattatcgacgagcgcctgatcaaccccgacggctccctgctgttccgagtaaccatcaacggagtgaccggctggcggctgtgcgaacgcattctggcgtaaacactcactccacaacccaagaatctgcagctaacttattttcccctagctttccccagacaccctgttttattttattataatgaattttgtttgttgatgtgaaacattatgccttaagtaatgttaattcttatttaagttattgatgttttaagtttatctttcatggtactagtgttttttagatacagagacttggggaaattgcttttcctcttgaaccacagttctacccctgggatgttttgagggtctttgcaagaatcattaatacaaagaattttttttaacattccaatgcattgctaaaatattattgtggaaatgaatattttgtaactattacaccaaataaatatatttttgtaca

SEQ ID NO: 67 - DNA, 1013 bp, Artificial Sequence
  Synthetic
gaggaaccgagaggctgagactaacccagaaacatccaattctcaaactgaagctcgcactctcgcctccagcatgtggcagattgttttctttactctgagctgtgatcttgtcttggccgcagccgtcttcacactcgaagatttcgttggggactggcgacagacagccggctacaacctggaccaagtccttgaacagggaggtgtgtccagtttgtttcagaatctcggggtgtccgtaactccgatccaaaggattgtcctgagcggtgaaaatgggctgaagatcgacatccatgtcatcatcccgtatgaaggtctgagcggcgaccaaatgggccagatcgaaaaaatttttaaggtggtgtaccctgtggatgatcatcactttaaggtgatcctgcactatggcacactggtaatcgacggggttacgccgaacatgatcgactatttcggacggccgtatgaaggcatcgccgtgttcgacggcaaaaagatcactgtaacagggaccctgtggaacggcaacaaaattatcgacgagcgcctgatcaaccccgacggctccctgctgttccgagtaaccatcaacggagtgaccggctggcggctgtgcgaacgcattctggcgtaaacactcactccacaacccaagaatctgcagctaacttattttcccctagctttccccagacaccctgttttattttattataatgaattttgtttgttgatgtgaaacattatgccttaagtaatgttaattcttatttaagttattgatgttttaagtttatctttcatggtactagtgttttttagatacagagacttggggaaattgcttttcctcttgaaccacagttctacccctgggatgttttgagggtctttgcaagaatcattaatacaaagaattttttttaacattccaatgcattgctaaaatattattgtggaaatgaatattttgtaactattacaccaaataaatatatttttgtaca

SEQ ID NO: 68 - DNA, 962 bp, Artificial Sequence
  Synthetic
gaggaaccgagaggctgagactaacccagaaacatccaattctcaaactgaagctcgcactctcgcctccagcatggtcttcacactcgaagatttcgttggggactggcgacagacagccggctacaacctggaccaagtccttgaacagggaggtgtgtccagtttgtttcagaatctcggggtgtccgtaactccgatccaaaggattgtcctgagcggtgaaaatgggctgaagatcgacatccatgtcatcatcccgtatgaaggtctgagcggcgaccaaatgggccagatcgaaaaaatttttaaggtggtgtaccctgtggatgatcatcactttaaggtgatcctgcactatggcacactggtaatcgacggggttacgccgaacatgatcgactatttcggacggccgtatgaaggcatcgccgtgttcgacggcaaaaagatcactgtaacagggaccctgtggaacggcaacaaaattatcgacgagcgcctgatcaaccccgacggctccctgctgttccgagtaaccatcaacggagtgaccggctggcggctgtgcgaacgcattctggcgtaaacactcactccacaacccaagaatctgcagctaacttattttcccctagctttccccagacaccctgttttattttattataatgaattttgtttgttgatgtgaaacattatgccttaagtaatgttaattcttatttaagttattgatgttttaagtttatctttcatggtactagtgttttttagatacagagacttggggaaattgcttttcctcttgaaccacagttctacccctgggatgttttgagggtctttgcaagaatcattaatacaaagaattttttttaacattccaatgcattgctaaaatattattgtggaaatgaatattttgtaactattacaccaaataaatatatttttgtaca

SEQ ID NO: 69 - DNA, 1198 bp, Artificial Sequence
  Synthetic
ataaaagcccaggggcaagcggtccggataacggctagcctgaggagctgctgcgacagtccactacctttttcgagagtgactcccgttgtcccaaggcttcccagagcgaacctgtgcggctgcaggcaccggcgcgtcgagtttccggcgtccggaaggaccgagctcttctcgcgaatccagtgttccgtttccagcccccaatctcagagcggagccgacagagagcagggaaccggcatgaaagtctctgccgcccttctgtgcctgctgctcatagcagccaccttcattccccaagggctcgctgtcttcacactcgaagatttcgttggggactggcgacagacagccggctacaacctggaccaagtccttgaacagggaggtgtgtccagtttgtttcagaatctcggggtgtccgtaactccgatccaaaggattgtcctgagcggtgaaaatgggctgaagatcgacatccatgtcatcatcccgtatgaaggtctgagcggcgaccaaatgggccagatcgaaaaaatttttaaggtggtgtaccctgtggatgatcatcactttaaggtgatcctgcactatggcacactggtaatcgacggggttacgccgaacatgatcgactatttcggacggccgtatgaaggcatcgccgtgttcgacggcaaaaagatcactgtaacagggaccctgtggaacggcaacaaaattatcgacgagcgcctgatcaaccccgacggctccctgctgttccgagtaaccatcaacggagtgaccggctggcggctgtgcgaacgcattctggcgtaaacactcactccacaacccaagaatctgcagctaacttattttcccctagctttccccagacaccctgttttattttattataatgaattttgtttgttgatgtgaaacattatgccttaagtaatgttaattcttatttaagttattgatgttttaagtttatctttcatggtactagtgttttttagatacagagacttggggaaattgcttttcctcttgaaccacagttctacccctgggatgttttgagggtctttgcaagaatcattaatacaaagaattttttttaacattccaatgcattgctaaaatattattgtggaaatgaatattttgtaactattacaccaaataaatatatttttgtaca

SEQ ID NO: 70 - DNA, 1067 bp, Artificial Sequence
  Synthetic
catatcttcattcttcactctttccccccccccccttatcctcctatctaatcctctcatctctctcctcctcttcctccaacaacaactaacaatggcagcaactacaacaatgaaagtctctgccgcccttctgtgcctgctgctcatagcagccaccttcattccccaagggctcgctgtcttcacactcgaagatttcgttggggactggcgacagacagccggctacaacctggaccaagtccttgaacagggaggtgtgtccagtttgtttcagaatctcggggtgtccgtaactccgatccaaaggattgtcctgagcggtgaaaatgggctgaagatcgacatccatgtcatcatcccgtatgaaggtctgagcggcgaccaaatgggccagatcgaaaaaatttttaaggtggtgtaccctgtggatgatcatcactttaaggtgatcctgcactatggcacactggtaatcgacggggttacgccgaacatgatcgactatttcggacggccgtatgaaggcatcgccgtgttcgacggcaaaaagatcactgtaacagggaccctgtggaacggcaacaaaattatcgacgagcgcctgatcaaccccgacggctccctgctgttccgagtaaccatcaacggagtgaccggctggcggctgtgcgaacgcattctggcgtaaacactcactccacaacccaagaatctgcagctaacttattttcccctagctttccccagacaccctgttttattttattataatgaattttgtttgttgatgtgaaacattatgccttaagtaatgttaattcttatttaagttattgatgttttaagtttatctttcatggtactagtgttttttagatacagagacttggggaaattgcttttcctcttgaaccacagttctacccctgggatgttttgagggtctttgcaagaatcattaatacaaagaattttttttaacattccaatgcattgctaaaatattattgtggaaatgaatattttgtaactattacaccaaataaatatatttttgtaca

SEQ ID NO: 71 - DNA, 1052 bp, Artificial Sequence
  Synthetic
aaagtgattgattcggatactgacactgtaggatctggggagagaggaacaaaggaccgtgaaagctgctctgtaaaagctgacacagccctcccaagtgagcaggactgttcttcccactgcaatctgacagtttactgcatgcctggagagaacacagcagtaaaaaccaggtttgctactggaaaaagaggaaagagaagactttcattgacggacccagccatggcagcgtagcagccctgcgttttagacggcagcagctcgggactctggacgtgtgtttgccctcaagtttgctaagctgctggtttattactgaagaaagaatgaaagtctctgccgcccttctgtgcctgctgctcatagcagccaccttcattccccaagggctcgctgtcttcacactcgaagatttcgttggggactggcgacagacagccggctacaacctggaccaagtccttgaacagggaggtgtgtccagtttgtttcagaatctcggggtgtccgtaactccgatccaaaggattgtcctgagcggtgaaaatgggctgaagatcgacatccatgtcatcatcccgtatgaaggtctgagcggcgaccaaatgggccagatcgaaaaaatttttaaggtggtgtaccctgtggatgatcatcactttaaggtgatcctgcactatggcacactggtaatcgacggggttacgccgaacatgatcgactatttcggacggccgtatgaaggcatcgccgtgttcgacggcaaaaagatcactgtaacagggaccctgtggaacggcaacaaaattatcgacgagcgcctgatcaaccccgacggctccctgctgttccgagtaaccatcaacggagtgaccggctggcggctgtgcgaacgcattctggcgtaaggctgctgcagctgcatgggtgcctgctgctgcctgccttggcctgatggccaggccagagtgctgccagtcctctgcatgttctgctcttgtgcccttctgagcccacaataaaggctgagctcttatcttgcaaaaggc

SEQ ID NO: 72 - DNA, 1064 bp, Artificial Sequence
  Synthetic
aaagtgattgattcggatactgacactgtaggatctggggagagaggaacaaaggaccgtgaaagctgctctgtaaaagctgacacagccctcccaagtgagcaggactgttcttcccactgcaatctgacagtttactgccctggagagaacacagcagtaaaaaccaggtttgctactggaaaaagaggaaagagaagactttcattgacggacccagccgcagcgtagcagccctgcgttttagacggcagcagctcgggactctggacgtgtgtttgccctcaagtttgctaagctgctggtttattactgaagaaagaatgaactccttctccacaagcgccttcggtccagttgccttctccctgggcctgctcctggtgttgcctgctgccttccctgccccagtcttcacactcgaagatttcgttggggactggcgacagacagccggctacaacctggaccaagtccttgaacagggaggtgtgtccagtttgtttcagaatctcggggtgtccgtaactccgatccaaaggattgtcctgagcggtgaaaatgggctgaagatcgacatccatgtcatcatcccgtatgaaggtctgagcggcgaccaaatgggccagatcgaaaaaatttttaaggtggtgtaccctgtggatgatcatcactttaaggtgatcctgcactatggcacactggtaatcgacggggttacgccgaacatgatcgactatttcggacggccgtatgaaggcatcgccgtgttcgacggcaaaaagatcactgtaacagggaccctgtggaacggcaacaaaattatcgacgagcgcctgatcaaccccgacggctccctgctgttccgagtaaccatcaacggagtgaccggctggcggctgtgcgaacgcattctggcgtaaggctgctgcagctgcatgggtgcctgctgctgcctgccttggcctgatggccaggccagagtgctgccagtcctctgcatgttctgctcttgtgcccttctgagcccacaataaaggctgagctcttatcttgcaaaaggc

SEQ ID NO: 73 - DNA, 1034 bp, Artificial Sequence
  Synthetic
aaagtgattgattcggatactgacactgtaggatctggggagagaggaacaaaggaccgtgaaagctgctctgtaaaagctgacacagccctcccaagtgagcaggactgttcttcccactgcaatctgacagtttactgcatgcctggagagaacacagcagtaaaaaccaggtttgctactggaaaaagaggaaagagaagactttcattgacggacccagccatggcagcgtagcagccctgcgttttagacggcagcagctcgggactctggacgtgtgtttgccctcaagtttgctaagctgctggtttattactgaagaaagaatgggagtgaaagttctttttgcccttatttgtattgctgtggccgaggccgtcttcacactcgaagatttcgttggggactggcgacagacagccggctacaacctggaccaagtccttgaacagggaggtgtgtccagtttgtttcagaatctcggggtgtccgtaactccgatccaaaggattgtcctgagcggtgaaaatgggctgaagatcgacatccatgtcatcatcccgtatgaaggtctgagcggcgaccaaatgggccagatcgaaaaaatttttaaggtggtgtaccctgtggatgatcatcactttaaggtgatcctgcactatggcacactggtaatcgacggggttacgccgaacatgatcgactatttcggacggccgtatgaaggcatcgccgtgttcgacggcaaaaagatcactgtaacagggaccctgtggaacggcaacaaaattatcgacgagcgcctgatcaaccccgacggctccctgctgttccgagtaaccatcaacggagtgaccggctggcggctgtgcgaacgcattctggcgtaaggctgctgcagctgcatgggtgcctgctgctgcctgccttggcctgatggccaggccagagtgctgccagtcctctgcatgttctgctcttgtgcccttctgagcccacaataaaggctgagctcttatcttgcaaaaggc

SEQ ID NO: 74 - DNA, 842 bp, Artificial Sequence
  Synthetic
catatcttcattcttcactctttccccccccccccttatcctcctatctaatcctctcatctctctcctcctcttcctccaacaacaactaacaatggcagcaactacaacaatgaaagtctctgccgcccttctgtgcctgctgctcatagcagccaccttcattccccaagggctcgctgtcttcacactcgaagatttcgttggggactggcgacagacagccggctacaacctggaccaagtccttgaacagggaggtgtgtccagtttgtttcagaatctcggggtgtccgtaactccgatccaaaggattgtcctgagcggtgaaaatgggctgaagatcgacatccatgtcatcatcccgtatgaaggtctgagcggcgaccaaatgggccagatcgaaaaaatttttaaggtggtgtaccctgtggatgatcatcactttaaggtgatcctgcactatggcacactggtaatcgacggggttacgccgaacatgatcgactatttcggacggccgtatgaaggcatcgccgtgttcgacggcaaaaagatcactgtaacagggaccctgtggaacggcaacaaaattatcgacgagcgcctgatcaaccccgacggctccctgctgttccgagtaaccatcaacggagtgaccggctggcggctgtgcgaacgcattctggcgtaattttgagtaattttcaattttgtttttgtttttgtttttgttgttgggagttgttgtaatttggtaaatgttggggtcactaaaatcttttgttgcaattttagcacctttttattagatatataaaattgggtttagatgtagttaa

SEQ ID NO: 75 - DNA, 824 bp, Artificial Sequence
  Synthetic
catatcttcattcttcactctttccccccccccccttatcctcctatctaatcctctcatctctctcctcctcttcctccaacaacaactaacaatgaaagtctctgccgcccttctgtgcctgctgctcatagcagccaccttcattccccaagggctcgctgtcttcacactcgaagatttcgttggggactggcgacagacagccggctacaacctggaccaagtccttgaacagggaggtgtgtccagtttgtttcagaatctcggggtgtccgtaactccgatccaaaggattgtcctgagcggtgaaaatgggctgaagatcgacatccatgtcatcatcccgtatgaaggtctgagcggcgaccaaatgggccagatcgaaaaaatttttaaggtggtgtaccctgtggatgatcatcactttaaggtgatcctgcactatggcacactggtaatcgacggggttacgccgaacatgatcgactatttcggacggccgtatgaaggcatcgccgtgttcgacggcaaaaagatcactgtaacagggaccctgtggaacggcaacaaaattatcgacgagcgcctgatcaaccccgacggctccctgctgttccgagtaaccatcaacggagtgaccggctggcggctgtgcgaacgcattctggcgtaattttgagtaattttcaattttgtttttgtttttgtttttgttgttgggagttgttgtaatttggtaaatgttggggtcactaaaatcttttgttgcaattttagcacctttttattagatatataaaattgggtttagatgtagttaa

SEQ ID NO: 76 - DNA, 809 bp, Artificial Sequence
  Synthetic
catatcttcattcttcactctttccccccccccccttatcctcctatctaatcctctcatctctctcctcctcttcctccaacaacaactaacaatgtggcagattgttttctttactctgagctgtgatcttgtcttggccgcagccgtcttcacactcgaagatttcgttggggactggcgacagacagccggctacaacctggaccaagtccttgaacagggaggtgtgtccagtttgtttcagaatctcggggtgtccgtaactccgatccaaaggattgtcctgagcggtgaaaatgggctgaagatcgacatccatgtcatcatcccgtatgaaggtctgagcggcgaccaaatgggccagatcgaaaaaatttttaaggtggtgtaccctgtggatgatcatcactttaaggtgatcctgcactatggcacactggtaatcgacggggttacgccgaacatgatcgactatttcggacggccgtatgaaggcatcgccgtgttcgacggcaaaaagatcactgtaacagggaccctgtggaacggcaacaaaattatcgacgagcgcctgatcaaccccgacggctccctgctgttccgagtaaccatcaacggagtgaccggctggcggctgtgcgaacgcattctggcgtaattttgagtaattttcaattttgtttttgtttttgtttttgttgttgggagttgttgtaatttggtaaatgttggggtcactaaaatcttttgttgcaattttagcacctttttattagatatataaaattgggtttagatgtagttaa

SEQ ID NO: 77 - DNA, 1083 bp, Artificial Sequence
  Synthetic
ataaaagcccaggggcaagcggtccggataacggctagcctgaggagctgctgcgacagtccactacctttttcgagagtgactcccgttgtcccaaggcttcccagagcgaacctgtgcggctgcaggcaccggcgcgtcgagtttccggcgtccggaaggaccgagctcttctcgcgaatccagtgttccgtttccagcccccaatctcagagcggagccgacagagagcagggaaccggcatgaaagtctctgccgcccttctgtgcctgctgctcatagcagccaccttcattccccaagggctcgctgtcttcacactcgaagatttcgttggggactggcgacagacagccggctacaacctggaccaagtccttgaacagggaggtgtgtccagtttgtttcagaatctcggggtgtccgtaactccgatccaaaggattgtcctgagcggtgaaaatgggctgaagatcgacatccatgtcatcatcccgtatgaaggtctgagcggcgaccaaatgggccagatcgaaaaaatttttaaggtggtgtaccctgtggatgatcatcactttaaggtgatcctgcactatggcacactggtaatcgacggggttacgccgaacatgatcgactatttcggacggccgtatgaaggcatcgccgtgttcgacggcaaaaagatcactgtaacagggaccctgtggaacggcaacaaaattatcgacgagcgcctgatcaaccccgacggctccctgctgttccgagtaaccatcaacggagtgaccggctggcggctgtgcgaacgcattctggcgtaagggcctttccaagattgctgtttttgttttggagcttcaagactttgcatttcctagtatttctgtttgtcagttctcaatttcctgtgtttgcaatgttgaaattttttggtgaagtactgaacttgctttttttccggtttctacatgcagagatgaatttatactgccatcttacgactatttcttctttttaatacacttaactcaggccattttttaagttggttacttcaaagtaaataaactttaaaattc

SEQ ID NO: 78 - DNA, 984 bp, Artificial Sequence
  Synthetic
gggctgggggagggtatataagccgagtaggcgacggtgaggtcgacgccggccaagacagcacagacagattgacctattggggtgtttcgcgagtgtgagagggaagcgccgcggcctgtatttctagacctgcccttcgcctggttcgtggcgccttgtgaccccgggcccctgccgcctgcaagtcggaaattgcgctgtgctcctgtgctacggcctgtggctggactgcctgctgctgcccaactggctggcaagatgaaagtctctgccgcccttctgtgcctgctgctcatagcagccaccttcattccccaagggctcgctgtcttcacactcgaagatttcgttggggactggcgacagacagccggctacaacctggaccaagtccttgaacagggaggtgtgtccagtttgtttcagaatctcggggtgtccgtaactccgatccaaaggattgtcctgagcggtgaaaatgggctgaagatcgacatccatgtcatcatcccgtatgaaggtctgagcggcgaccaaatgggccagatcgaaaaaatttttaaggtggtgtaccctgtggatgatcatcactttaaggtgatcctgcactatggcacactggtaatcgacggggttacgccgaacatgatcgactatttcggacggccgtatgaaggcatcgccgtgttcgacggcaaaaagatcactgtaacagggaccctgtggaacggcaacaaaattatcgacgagcgcctgatcaaccccgacggctccctgctgttccgagtaaccatcaacggagtgaccggctggcggctgtgcgaacgcattctggcgtaaggctgctgcagctgcatgggtgcctgctgctgcctgccttggcctgatggccaggccagagtgctgccagtcctctgcatgttctgctcttgtgcccttctgagcccacaataaaggctgagctcttatcttgcaaaaggc

SEQ ID NO: 79 - DNA, 898 bp, Artificial Sequence
  Synthetic
agctgttcttggctgacttcacatcaaaactcctatactgacctgagacagaggcagcagtgatacccacctgagagatcctgtgtttgaacaactgcttcccaaaacggaaagtatttcaagcctaaacctttgggtgaaaagaactcttgaagtcatgaactccttctccacaagcgccttcggtccagttgccttctccctgggcctgctcctggtgttgcctgctgccttccctgccccagtcttcacactcgaagatttcgttggggactggcgacagacagccggctacaacctggaccaagtccttgaacagggaggtgtgtccagtttgtttcagaatctcggggtgtccgtaactccgatccaaaggattgtcctgagcggtgaaaatgggctgaagatcgacatccatgtcatcatcccgtatgaaggtctgagcggcgaccaaatgggccagatcgaaaaaatttttaaggtggtgtaccctgtggatgatcatcactttaaggtgatcctgcactatggcacactggtaatcgacggggttacgccgaacatgatcgactatttcggacggccgtatgaaggcatcgccgtgttcgacggcaaaaagatcactgtaacagggaccctgtggaacggcaacaaaattatcgacgagcgcctgatcaaccccgacggctccctgctgttccgagtaaccatcaacggagtgaccggctggcggctgtgcgaacgcattctggcgtaaggctgctgcagctgcatgggtgcctgctgctgcctgccttggcctgatggccaggccagagtgctgccagtcctctgcatgttctgctcttgtgcccttctgagcccacaataaaggctgagctcttatcttgcaaaaggc

SEQ ID NO: 80 - DNA, 1060 bp, Artificial Sequence
  Synthetic
caagcttagcctggccgggaaacgggaggcgtggaggccgggagcagcccccggggtcatcgccctgccaccgccgcccgattgctttagcttggaaattccggagctgaagcggccagcgagggaggatgaccctctcggcccgggcaccctgtcagtccggaaataactgcagcatttgttccggaggggaaggcgcgaggtttccgggaaagcagcaccgccccttggcccccaggtggctagcgctataaaggatcacgcgccccagtcgacgctgagctcctctgctactcagagttgcaacctcagcctcgctatgaactccttctccacaagcgccttcggtccagttgccttctccctgggcctgctcctggtgttgcctgctgccttccctgccccagtcttcacactcgaagatttcgttggggactggcgacagacagccggctacaacctggaccaagtccttgaacagggaggtgtgtccagtttgtttcagaatctcggggtgtccgtaactccgatccaaaggattgtcctgagcggtgaaaatgggctgaagatcgacatccatgtcatcatcccgtatgaaggtctgagcggcgaccaaatgggccagatcgaaaaaatttttaaggtggtgtaccctgtggatgatcatcactttaaggtgatcctgcactatggcacactggtaatcgacggggttacgccgaacatgatcgactatttcggacggccgtatgaaggcatcgccgtgttcgacggcaaaaagatcactgtaacagggaccctgtggaacggcaacaaaattatcgacgagcgcctgatcaaccccgacggctccctgctgttccgagtaaccatcaacggagtgaccggctggcggctgtgcgaacgcattctggcgtaaggctgctgcagctgcatgggtgcctgctgctgcctgccttggcctgatggccaggccagagtgctgccagtcctctgcatgttctgctcttgtgcccttctgagcccacaataaaggctgagctcttatcttgcaaaaggc

SEQ ID NO: 81 - DNA, 1150 bp, Artificial Sequence
  Synthetic
gtctcaatattagagtctcaacccccaataaatataggactggagatgtctgaggctcattctgccctggagcccaccgggaacgaaagagaagctctatctcccctccaggagcccagctatgaactccttctccacaagcgccttcggtccagttgccttctccctggggctgctcctggtgttgcctgctgccttccctgccccagtcttcacactcgaagatttcgttggggactggcgacagacagccggctacaacctggaccaagtccttgaacagggaggtgtgtccagtttgtttcagaatctcggggtgtccgtaactccgatccaaaggattgtcctgagcggtgaaaatgggctgaagatcgacatccatgtcatcatcccgtatgaaggtctgagcggcgaccaaatgggccagatcgaaaaaatttttaaggtggtgtaccctgtggatgatcatcactttaaggtgatcctgcactatggcacactggtaatcgacggggttacgccgaacatgatcgactatttcggacggccgtatgaaggcatcgccgtgttcgacggcaaaaagatcactgtaacagggaccctgtggaacggcaacaaaattatcgacgagcgcctgatcaaccccgacggctccctgctgttccgagtaaccatcaacggagtgaccggctggcggctgtgcgaacgcattctggcgtaacatgggcacctcagattgttgttgttaatgggcattccttcttctggtcagaaacctgtccactgggcacagaacttatgttgttctctatggagaactaaaagtatgagcgttaggacactattttaattatttttaatttattaatatttaaatatgtgaagctgagttaatttatgtaagtcatatttatatttttaagaagtaccacttgaaacattttatgtattagttttgaaataataatggaaagtggctatgcagtttgaatatcctttgtttcagagccagatcatttcttggaaagtgtaggcttacctcaaataaatggctaacttatacatatttttaaagaaatatttatattgtatttatataatgtataaatggtttttataccaataaatggcattttaaaaaattcagcaa

SEQ ID NO: 82 - DNA, 975 bp, Artificial Sequence
  Synthetic
gtggcagctcacagctattgtggtgggaaagggagggtggttggtggatgtcacagcttgggctttatctcccccagcagtggggactccacagcccctgggctacataacagcaagacagtccggagctgtagcagacctgattgagcctttgcagcagctgagagcatggcctagggtgggcggcaccattgtccagcagctgagtttcccagggaccttggagatagccgcagccctcatttgcaggggaagatgattcctgccagatttgccggggtgctgcttgctctggccctcattttgccagggaccctttgtgtcttcacactcgaagatttcgttggggactggcgacagacagccggctacaacctggaccaagtccttgaacagggaggtgtgtccagtttgtttcagaatctcggggtgtccgtaactccgatccaaaggattgtcctgagcggtgaaaatgggctgaagatcgacatccatgtcatcatcccgtatgaaggtctgagcggcgaccaaatgggccagatcgaaaaaatttttaaggtggtgtaccctgtggatgatcatcactttaaggtgatcctgcactatggcacactggtaatcgacggggttacgccgaacatgatcgactatttcggacggccgtatgaaggcatcgccgtgttcgacggcaaaaagatcactgtaacagggaccctgtggaacggcaacaaaattatcgacgagcgcctgatcaaccccgacggctccctgctgttccgagtaaccatcaacggagtgaccggctggcggctgtgcgaacgcattctggcgtaaggctgctgcagctgcatgggtgcctgctgctgcctgccttggcctgatggccaggccagagtgctgccagtcctctgcatgttctgctcttgtgcccttctgagcccacaataaaggctgagctcttatcttgcaaaaggc

SEQ ID NO: 83 - DNA, 497 bp, Homo sapiens
  5'UTR (1)..(497)
gccctaagccatcagcaatccttagtataggggcacactcatgcattcctgtcaagtcatcttgtgaaaggctgcctgcttccagcttggcttggatgtgcaaccttaataaaactcactgaggtctgggagaaaatagcagatctgcagcagatagggtagaggaaagggtctagaatatgtacacgcagctgactcaggcaggctccatgctgaacggtcacacagagaggaaacaataaatctcagctactatgcaataaatatctcaagttttaacgaagaaaaacatcattgcagtgaaataaaaaattttaaaattttagaacaaagctaacaaatggctagttttctatgattcttcttcaaacgctttctttgagggggaaagagtcaaacaaacaagcagttttacctgaaataaagaactagttttagaggtcagaagaaaggagcaagttttgcgagaggcacggaaggagtgtgctggcagtaca

SEQ ID NO: 84 - DNA, 45 bp, Homo sapiens
  sig_peptide (1)..(45)
atgacagttttcctttcctttgctttcctcgctgccattctgact

SEQ ID NO: 85 - protein, 15 aa, Homo sapiens
  SIGNAL (1)..(15)
MTVFLSFAFLAAILT

SEQ ID NO: 86 - DNA, 1452 bp, Homo sapiens
  CDS (1)..(1452)
cacatagggtgcagcaatcagcgccgaagtccagaaaacagtgggagaagatataaccggattcaacatgggcaatgtgcctacactttcattcttccagaacacgatggcaactgtcgtgagagtacgacagaccagtacaacacaaacgctctgcagagagatgctccacacgtggaaccggatttctcttcccagaaacttcaacatctggaacatgtgatggaaaattatactcagtggctgcaaaaacttgagaattacattgtggaaaacatgaagtcggagatggcccagatacagcagaatgcagttcagaaccacacggctaccatgctggagataggaaccagcctcctctctcagactgcagagcagaccagaaagctgacagatgttgagacccaggtactaaatcaaacttctcgacttgagatacagctgctggagaattcattatccacctacaagctagagaagcaacttcttcaacagacaaatgaaatcttgaagatccatgaaaaaaacagtttattagaacataaaatcttagaaatggaaggaaaacacaaggaagagttggacaccttaaaggaagagaaagagaaccttcaaggcttggttactcgtcaaacatatataatccaggagctggaaaagcaattaaacagagctaccaccaacaacagtgtccttcagaagcagcaactggagctgatggacacagtccacaaccttgtcaatctttgcactaaagaaggtgttttactaaagggaggaaaaagagaggaagagaaaccatttagagactgtgcagatgtatatcaagctggttttaataaaagtggaatctacactatttatattaataatatgccagaacccaaaaaggtgttttgcaatatggatgtcaatgggggaggttggactgtaatacaacatcgtgaagatggaagtctagatttccaaagaggctggaaggaatataaaatgggttttggaaatccctccggtgaatattggctggggaatgagtttatttttgccattaccagtcagaggcagtacatgctaagaattgagttaatggactgggaagggaaccgagcctattcacagtatgacagattccacataggaaatgaaaagcaaaactataggttgtatttaaaaggtcacactgggacagcaggaaaacagagcagcctgatcttacacggtgctgatttcagcactaaagatgctgataatgacaactgtatgtgcaaatgtgccctcatgttaacaggaggatggtggtttgatgcttgtggcccctccaatctaaatggaatgttctatactgcgggacaaaaccatggaaaactgaatgggataaagtggcactacttcaaagggcccagttactccttacgttccacaactatgatgattcgacctttagatttttga

SEQ ID NO: 87 - protein, 483 aa, Homo sapiens
HIGCSNQRRSPENSGRRYNRIQHGQCAYTFILPEHDGNCRESTTDQYNTNALQRDAPHVEPDFSSQKLQHLEHVMENYTQWLQKLENYIVENMKSEMAQIQQNAVQNHTATMLEIGTSLLSQTAEQTRKLTDVETQVLNQTSRLEIQLLENSLSTYKLEKQLLQQTNEILKIHEKNSLLEHKILEMEGKHKEELDTLKEEKENLQGLVTRQTYIIQELEKQLNRATTNNSVLQKQQLELMDTVHNLVNLCTKEGVLLKGGKREEEKPFRDCADVYQAGFNKSGIYTIYINNMPEPKKVFCNMDVNGGGWTVIQHREDGSLDFQRGWKEYKMGFGNPSGEYWLGNEFIFAITSQRQYMLRIELMDWEGNRAYSQYDRFHIGNEKQNYRLYLKGHTGTAGKQSSLILHGADFSTKDADNDNCMCKCALMLTGGWWFDACGPSNLNGMFYTAGQNHGKLNGIKWHYFKGPSYSLRSTTMMIRPLDF

SEQ ID NO: 88 - DNA, 2373 bp, Homo sapiens
  5'UTR (1)..(2373)
aagcgcaatgtcagaagcgattatgaaagcaacaaagaaatccggagaagctgccaggtgagaaactgtttgaaaacttcagaagcaaacaatattgtctcccttccagcaataagtggtagttatgtgaagtcaccaaggttcttgaccgtgaatctggagccgtttgagttcacaagagtctctacttggggtgacagtgctcacgtggctcgactatagaaaactccactgactgtcgggctttaaaaagggaagaaactgctgagcttgctgtgcttcaaactactactggaccttattttggaactatggtagccagatgataaatatggttaatttcatgtaaaacagaaaaaaagagtgaaaaagagaatatacatgaagaatagaaacaagcctgccataatcctttggaaaagatgtattataccagtgaaaaggtgttatatctatgcaaacctactaacaaattatactgttgcacaattttgataaaaatttagaacagcattgtcctctgagttggttaaatgttaatggatttcagaagcctaattccagtatcatacttactagttgatttctgcttacccatcttcaaatgaaaattccatttttgtaagccataatgaactgtagtacatggacaataagtgtgtggtagaaacaaactccattactctgatttttgatacagttttcagaaaaagaaatgaacataatcaagtaaggatgtatgtggtgaaaacttaccacccccatactatggttttcatttactctaaaaactgattgaatgatatataaatatatttatagcctgagtaaagttaaaagaatgtaaaatatatcatcaagttcttaaaataatatacatgcatttaatatttcctttgatattatacaggaaagcaatattttggagtatgttaagttgaagtaaaagcaagtactctggagcagttcattttacagtatctacttgcatgtgtatacatacatgtaacttcattattttaaaaatatttttagaactccaatactcaccctgttatgtcttgctaatttaaattttgctaattaactgaaacatgcttaccagattcacactgttccagtgtctataaaagaaacactttgaagtctataaaaaataaaataattataaatatcattgtacatagcatgtttatatctgcaaaaaacctaatagctaattaatctggaatatgcaacattgtccttaattgatgcaaataacacaaatgctcaaagaaatctactatatcccttaatgaaatacatcattcttcatatatttctccttcagtccattcccttaggcaatttttaatttttaaaaattattatcaggggagaaaaattggcaaaactattatatgtaagggaaatatatacaaaaagaaaattaatcatagtcacctgactaagaaattctgactgctagttgccataaataactcaatggaaatattcctatgggataatgtattttaagtgaatttttggggtgcttgaagttactgcattattttatcaagaagtcttctctgcctgtaagtgtccaaggttatgacagtaaacagtttttattaaaacatgagtcactatgggatgagaaaattgaaataaagctactgggcctcctctcataaaagagacagttgttggcaaggtagcaataccagtttcaaacttggtgacttgatccactatgccttaatggtttcctccatttgagaaaataaagctattcacattgttaagaaaaatactttttaaagtttaccatcaagtcttttttatatttatgtgtctgtattctacccctttttgccttacaagtgatatttgcaggtattataccatttttctattcttggtggcttcttcatagcaggtaagcctctccttctaaaaacttctcaactgttttcatttaagggaaagaaaatgagtattttgtccttttgtgttcctacagacactttcttaaaccagtttttggataaagaatactatttccaaactcatattacaaaaacaaaataaaataataaaaaaagaaagcatgatatttactgttttgttgtctgggtttgagaaatgaaatattgtttccaattatttataataaatcagtataaaatgttttatgattgttatgtgtattatgtaatacgtacatgtttatggcaatttaacatgtgtattcttttaattgtttcagaataggataattaggtattcgaattttgtctttaaaattcatgtggtttctatgcaaagttcttcatatcatcacaacattatttgatttaaataaaattgaaagtaatatttgtgcaa

SEQ ID NO: 89 - DNA, 120 bp, Homo sapiens
  5'UTR (1)..(120)
agacagaggtttgtagctgcagctgcaggcaagcctggccactgttggctgcagcaggacatcccaggcacagcccctagggctctgagcagacatccctcgccattgacacatcttcag

SEQ ID NO: 90 - DNA, 66 bp, Homo sapiens
  sig_peptide (1)..(66)
atgctctcccagctagccatgctgcagggcagcctcctccttgtggttgccaccatgtctgtggct

SEQ ID NO: 91 - protein, 22 aa, Homo sapiens
  SIGNAL (1)..(22)
MLSQLAMLQGSLLLVVATMSVA

SEQ ID NO: 92 - DNA, 1446 bp, Homo sapiens
  CDS (1)..(1446)
caacagacaaggcaggaggcggataggggctgcgagacacttgtagtccagcacggccactgtagctacaccttcttgctgcccaagtctgagccctgccctccggggcctgaggtctccagggactccaacaccctccagagagaatcactggccaacccactgcacctggggaagttgcccacccagcaggtgaaacagctggagcaggcactgcagaacaacacgcagtggctgaagaagctagagagggccatcaagacgatcttgaggtcgaagctggagcaggtccagcagcaaatggcccagaatcagacggcccccatgctagagctgggcaccagcctcctgaaccagaccactgcccagatccgcaagctgaccgacatggaggctcagctcctgaaccagacatcaagaatggatgcccagatgccagagacctttctgtccaccaacaagctggagaaccagctgctgctacagaggcagaagctccagcagcttcagggccaaaacagcgcgctcgagaagcggttgcaggccctggagaccaagcagcaggaggagctggccagcatcctcagcaagaaggcgaagctgctgaacacgctgagccgccagagcgccgccctcaccaacatcgagcgcggcctgcgcggtgtcaggcacaactccagcctcctgcaggaccagcagcacagcctgcgccagctgctggtgttgttgcggcacctggtgcaagaaagggctaacgcctcggccccggccttcataatggcaggtgagcaggtgttccaggactgtgcagagatccagcgctctggggccagtgccagtggtgtctacaccatccaggtgtccaatgcaacgaagcccaggaaggtgttctgtgacctgcagagcagtggaggcaggtggaccctcatccagcgccgtgagaatggcaccgtgaattttcagcggaactggaaggattacaaacagggcttcggagacccagctggggagcactggctgggcaatgaagtggtgcaccagctcaccagaagggcagcctactctctgcgtgtggagctgcaagactgggaaggccacgaggcctatgcccagtacgaacatttccacctgggcagtgagaaccagctatacaggctttctgtggtcgggtacagcggctcagcagggcgccagagcagcctggtcctgcagaacaccagctttagcacccttgactcagacaacgaccactgtctctgcaagtgtgcccaagtgatgtctggagggtggtggtttgacgcctgtggcctgtcaaacctcaacggcgtctactaccacgctcccgacaacaagtacaagatggacggcatccgctggcactacttcaagggccccagctactcactgcgtgcctctcgcatgatgatacggcctttggacatctaa

SEQ ID NO: 93 - protein, 481 aa, Homo sapiens
QQTRQEADRGCETLVVQHGHCSYTFLLPKSEPCPPGPEVSRDSNTLQRESLANPLHLGKLPTQQVKQLEQALQNNTQWLKKLERAIKTILRSKLEQVQQQMAQNQTAPMLELGTSLLNQTTAQIRKLTDMEAQLLNQTSRMDAQMPETFLSTNKLENQLLLQRQKLQQLQGQNSALEKRLQALETKQQEELASILSKKAKLLNTLSRQSAALTNIERGLRGVRHNSSLLQDQQHSLRQLLVLLRHLVQERANASAPAFIMAGEQVFQDCAEIQRSGASASGVYTIQVSNATKPRKVFCDLQSSGGRWTLIQRRENGTVNFQRNWKDYKQGFGDPAGEHWLGNEVVHQLTRRAAYSLRVELQDWEGHEAYAQYEHFHLGSENQLYRLSVVGYSGSAGRQSSLVLQNTSFSTLDSDNDHCLCKCAQVMSGGWWFDACGLSNLNGVYYHAPDNKYKMDGIRWHYFKGPSYSLRASRMMIRPLDI

SEQ ID NO: 94 - DNA, 3061 bp, Homo sapiens
  3'UTR (1)..(3061)
cgagcagctgtgccagaggctggaccacacaggagaagctcggacttggcactcctggacaacctggacccagatgcaagacactgtgccaccgccttccctgacaccctgggcttcctgagccagccctccttgacccagaagtccagaagggtcatctgccccccaactcccctccgtctgtgacatggagggtgttcggggcccatccctctgatgtagtcctcgcccctcttctctccctcccccttcaggggctccctgcctgagggtcacagtaccttgaatgggctgagaacagaccaaacttgattcccatgaccaatggtggggttgcaggcaggtgggaatgtatttgcacatcggaagctgcccagatggcccaggttctctcccttggattggcaagaaggccatctcccattctaagctcctgttccaagattttctagtcttgagatgtccttgaactttcttttcaagtctgaaggggctgcatccaccccttagtgggtgggttaatcattatttccccttcacacttcaccacttctaggttctaatgaccctagatctcagggtctttagacttcaccacttctaggctttaccacttcaccacttctaggctccaatgtttggagctcagggtctttaggagacccaaaaggacatgctccttcacctccagcatgtcctagaggatgtgtcacagggaataactatggcttgtctctaaaagtacctatgagcaatgagaaaaggaaacagcaggttaagtcaaagtgaacaggcactcttcactgcaggactgatcagagcctttaatatggccaagtgccttgtgactacccatgaaggggctagagtgggcagctttctccaaatttacttatttgaaaatgggctcggtttgtcccagagcatctcacaggactgtagatgctcttggacaaagctagtgctcccctggcataaggaggagccctacgaccccatccccaccccagctatactcaccctttttggctacaagggccacagtgacagcctcaaacaacctctaaaaacaactggaaataacctttcagttaaaacagataccatccctgaagaagggtctagaactaggtccctgtctgtgttataggctcatgtcctccaaggctccttcaagtcccaggaagctgatctctacctgggtggcttcccttaggactccctgtaacctcaactcccccaggctcaattacagggactgttaggcaggacatctgtctccaagtccagatcctctctgcctccaagccctaacccctagcctccctcccttccccatccagcagtgatgctgcctctgtggtggtaggtggggagctgcaggggaggagataaggcctctgcctgagtttgggagaccagggccctcatagcttctttcagaggatggagtcagaaaggatccacagctactctgtcacctgcccccatcactgtgtcatgctgtctgccctgttgtcatcagccaacacccaggcatagccaggagcccacctgccctaccgccaggatacacctctgtcctcagaaggttttctcctggatgagactgagccaatgggaatgggaccccttcatccccctggctcgccccagccctgagtcccactctcagccgatccctgagtaaacccagcacagactgactttgatctcattcctgggaattagcactcttccccttcaagactcaaaggacatggttgctaatggtggcatttcaggcatgatgggaaatctttaggggcagattgctgcccagagagctcaaatcgccttaagcagcatttgcccagcagacctttatttagcctctactgtgtgcagtgtggtgtggtgggcagggctttggagtcggacaaacctgctccagctctgacactttggtccagtggctcagcctctcaaggcaccagttatcttcacatcatcaaagcctcagttttcccatctgtaaaatggagatgataatattccttcctggctgggctatggcaaggaggaaatgagaccatgtatgtcatcttcttaatagagcctggcatgaagcaggtgcctaataaatgtttgtcctcaaagaggagaatggggtgaggaaggcattccccagcacatgccgccccttctcctgcactcaggtgaggaaaaggcattttatttttgtatccacatcatttatttttctattgtagtttctaggctgactgcaagctagagaggagacagggcaaagctgtgaggcccagggacagaactcctctgggtgggttgaaggcccaagtccctctctactcccattttataagggggcaggaagctgatttgagttatcctcagacacctgttctttatgtaattttattttatttttttgagacagagtctcactctgtcacccaggctggagtgcagtggcatgatctcagatcactgcaatctctgcctcctggttcaagtgattctcctacctcagcctcctgagtaatgggattacagacgcctaccaccacgcccggaaaacttttgtatttttagtagaaacgggttttcaccatgttggccaggctggtctcaaactcctggcctcatgtgatccacctgcctcagcctcccaaagtgctgggattacaggcatgagccaccatacccagcctcagacacctgttcttaaatattcatccttctttcttaccttccttcctcttccatgccaggactcaggtataagggatagaaattctagccctaaggaataaattgactcacataactggaaagtctaagggtaaaggcaagtgaggttagatccagaggctcaaatgatgtcagctccacctctcagcccctccatctgccccgttgacttcattctcagccaggatctttcctcacaagaaggctctggcagccccaggctcatgtcctcccagctcagcatccctgacccggggagctccctcgtctccatgattccagtaaaggaatgattttctgcagccag

SEQ ID NO: 95 - DNA, 867 bp, Artificial Sequence
  Synthetic
  CDS (1)..(867)
gggatcttagacctagccccacagatgcttcgagaactccaggagactaatgcggcgctgcaagacgtgagagagctcttgcgacagcaggtcaaggagatcaccttcctgaagaatacggtgatggaatgtgacgcttgcggaggctcccttgtcaatctttgcactaaagaaggtgttttactaaagggaggaaaaagagaggaagagaaaccatttagagactgtgcagatgtatatcaagctggttttaataaaagtggaatctacactatttatattaataatatgccagaacccaaaaaggtgttttgcaatatggatgtcaatgggggaggttggactgtaatacaacatcgtgaagatggaagtctagatttccaaagaggctggaaggaatataaaatgggttttggaaatccctccggtgaatattggctggggaatgagtttatttttgccattaccagtcagaggcagtacatgctaagaattgagttaatggactgggaagggaaccgagcctattcacagtatgacagattccacataggaaatgaaaagcaaaactataggttgtatttaaaaggtcacactgggacagcaggaaaacagagcagcctgatcttacacggtgctgatttcagcactaaagatgctgataatgacaactgtatgtgcaaatgtgccctcatgttaacaggaggatggtggtttgatgcttgtggcccctccaatctaaatggaatgttctatactgcgggacaaaaccatggaaaactgaatgggataaagtggcactacttcaaagggcccagttactccttacgttccacaactatgatgattcgacctttagatttttga

SEQ ID NO: 96 - protein, 288 aa, Artificial Sequence
  Synthetic Construct
GILDLAPQMLRELQETNAALQDVRELLRQQVKEITFLKNTVMECDACGGSLVNLCTKEGVLLKGGKREEEKPFRDCADVYQAGFNKSGIYTIYINNMPEPKKVFCNMDVNGGGWTVIQHREDGSLDFQRGWKEYKMGFGNPSGEYWLGNEFIFAITSQRQYMLRIELMDWEGNRAYSQYDRFHIGNEKQNYRLYLKGHTGTAGKQSSLILHGADFSTKDADNDNCMCKCALMLTGGWWFDACGPSNLNGMFYTAGQNHGKLNGIKWHYFKGPSYSLRSTTMMIRPLDF

SEQ ID NO: 97 - DNA, 867 bp, Artificial Sequence
  Synthetic
  CDS (1)..(867)
gggatcttagacttgggcccgcagatgcttcgggaactgcaggaaaccaacgcggcgctgcaggacgtgcgggagctgctgcggcagcaggtcagggagatcacgttcctgaaaaacacggtgatggagtgtgacgcgtgcggaggctcccttgtcaatctttgcactaaagaaggtgttttactaaagggaggaaaaagagaggaagagaaaccatttagagactgtgcagatgtatatcaagctggttttaataaaagtggaatctacactatttatattaataatatgccagaacccaaaaaggtgttttgcaatatggatgtcaatgggggaggttggactgtaatacaacatcgtgaagatggaagtctagatttccaaagaggctggaaggaatataaaatgggttttggaaatccctccggtgaatattggctggggaatgagtttatttttgccattaccagtcagaggcagtacatgctaagaattgagttaatggactgggaagggaaccgagcctattcacagtatgacagattccacataggaaatgaaaagcaaaactataggttgtatttaaaaggtcacactgggacagcaggaaaacagagcagcctgatcttacacggtgctgatttcagcactaaagatgctgataatgacaactgtatgtgcaaatgtgccctcatgttaacaggaggatggtggtttgatgcttgtggcccctccaatctaaatggaatgttctatactgcgggacaaaaccatggaaaactgaatgggataaagtggcactacttcaaagggcccagttactccttacgttccacaactatgatgattcgacctttagatttttga

SEQ ID NO: 98 - protein, 288 aa, Artificial Sequence
  Synthetic Construct
GILDLGPQMLRELQETNAALQDVRELLRQQVREITFLKNTVMECDACGGSLVNLCTKEGVLLKGGKREEEKPFRDCADVYQAGFNKSGIYTIYINNMPEPKKVFCNMDVNGGGWTVIQHREDGSLDFQRGWKEYKMGFGNPSGEYWLGNEFIFAITSQRQYMLRIELMDWEGNRAYSQYDRFHIGNEKQNYRLYLKGHTGTAGKQSSLILHGADFSTKDADNDNCMCKCALMLTGGWWFDACGPSNLNGMFYTAGQNHGKLNGIKWHYFKGPSYSLRSTTMMIRPLDF

SEQ ID NO: 99 - DNA, 861 bp, Artificial Sequence
  Synthetic
gggatcttagaggaagacccggccgcctgcgagtccctggtgaaattccaagccaaagtggaggggctgctgcaggccctgaccaggaaactggaagctgtgagtaagcggctggccatcctggagaacacagttgtcggatcccttgtcaatcttgccactaaagaaggtgttttactaaagggaggaaaaagagaggaagagaaaccatttagagactgtgcagatgtatatcaagctggttttaataaaagtggaatctacactatttatattaataatatgccagaacccaaaaaggtgttttgcaatatggatgtcaatgggggaggttggactgtaatacaacatcgtgaagatggaagtctagatttccaaagaggctggaaggaatataaaatgggttttggaaatccctccggtgaatattggctggggaatgagtttatttttgccattaccagtcagaggcagtacatgctaagaattgagttaatggactgggaagggaaccgagcctattcacagtatgacagattccacataggaaatgaaaagcaaaactataggttgtatttaaaaggtcacactgggacagcaggaaaacagagcagcctgatcttacacggtgctgatttcagcactaaagatgctgataatgacaactgtatgtgcaaatgtgccctcatgttaacaggaggatggtggtttgatgcttgtggcccctccaatctaaatggaatgttctatactgcgggacaaaaccatggaaaactgaatgggataaagtggcactacttcaaagggcccagttactccttacgttccacaactatgatgattcgacctttagatttttga

SEQ ID NO: 100 - DNA, 870 bp, Artificial Sequence
  Synthetic
gggatcttagacctagccccacagatgcttcgagaactccaggagactaatgcggcgctgcaagacgtgagagagctcttgcgacagcaggtcaaggagatcaccttcctgaagaatacggtgatggaatgtgacgcttgcggaggctccttactgactatgatgtccacatcaaactcagctaaggaccccactgttgctaaagaagaacaaatcagcttcagagactgtgctgaagtattcaaatcaggacacaccacgaatggcatctacacgttaacattccctaattctacagaagagatcaaggcctactgtgacatggaagctggaggaggcgggtggacaattattcagcgacgtgaggatggcagcgttgattttcagaggacttggaaagaatataaagtgggatttggtaacccttcaggagaatattggctgggaaatgagtttgtttcgcaactgactaatcagcaacgctatgtgcttaaaatacaccttaaagactgggaagggaatgaggcttactcattgtatgaacatttctatctctcaagtgaagaactcaattataggattcaccttaaaggacttacagggacagccggcaaaataagcagcatcagccaaccaggaaatgattttagcacaaaggatggagacaacgacaaatgtatttgcaaatgttcacaaatgctaacaggaggctggtggtttgatgcatgtggtccttccaacttgaacggaatgtactatccacagaggcagaacacaaataagttcaacggcattaaatggtactactggaaaggctcaggctattcgctcaaggccacaaccatgatgatccgaccagcagatttctaa

SEQ ID NO: 101 - DNA, 3375 bp, Homo sapiens
  CDS (1)..(3375)
atggactctttagccagcttagttctctgtggagtcagcttgctcctttctggaactgtggaaggtgccatggacttgatcttgatcaattccctacctcttgtatctgatgctgaaacatctctcacctgcattgcctctgggtggcgcccccatgagcccatcaccataggaagggactttgaagccttaatgaaccagcaccaggatccgctggaagttactcaagatgtgaccagagaatgggctaaaaaagttgtttggaagagagaaaaggctagtaagatcaatggtgcttatttctgtgaagggcgagttcgaggagaggcaatcaggatacgaaccatgaagatgcgtcaacaagcttccttcctaccagctactttaactatgactgtggacaagggagataacgtgaacatatctttcaaaaaggtattgattaaagaagaagatgcagtgatttacaaaaatggttccttcatccattcagtgccccggcatgaagtacctgatattctagaagtacacctgcctcatgctcagccccaggatgctggagtgtactcggccaggtatataggaggaaacctcttcacctcggccttcaccaggctgatagtccggagatgtgaagcccagaagtggggacctgaatgcaaccatctctgtactgcttgtatgaacaatggtgtctgccatgaagatactggagaatgcatttgccctcctgggtttatgggaaggacgtgtgagaaggcttgtgaactgcacacgtttggcagaacttgtaaagaaaggtgcagtggacaagagggatgcaagtcttatgtgttctgtctccctgacccctatgggtgttcctgtgccacaggctggaagggtctgcagtgcaatgaagcatgccaccctggtttttacgggccagattgtaagcttaggtgcagctgcaacaatggggagatgtgtgatcgcttccaaggatgtctctgctctccaggatggcaggggctccagtgtgagagagaaggcataccgaggatgaccccaaagatagtggatttgccagatcatatagaagtaaacagtggtaaatttaatcccatttgcaaagcttctggctggccgctacctactaatgaagaaatgaccctggtgaagccggatgggacagtgctccatccaaaagactttaaccatacggatcatttctcagtagccatattcaccatccaccggatcctcccccctgactcaggagtttgggtctgcagtgtgaacacagtggctgggatggtggaaaagcccttcaacatttctgttaaagttcttccaaagcccctgaatgccccaaacgtgattgacactggacataactttgctgtcatcaacatcagctctgagccttactttggggatggaccaatcaaatccaagaagcttctatacaaacccgttaatcactatgaggcttggcaacatattcaagtgacaaatgagattgttacactcaactatttggaacctcggacagaatatgaactctgtgtgcaactggtccgtcgtggagagggtggggaagggcatcctggacctgtgagacgcttcacaacagcttctatcggactccctcctccaagaggtctaaatctcctgcctaaaagtcagaccactctaaatttgacctggcaaccaatatttccaagctcggaagatgacttttatgttgaagtggagagaaggtctgtgcaaaaaagtgatcagcagaatattaaagttccaggcaacttgacttcggtgctacttaacaacttacatcccagggagcagtacgtggtccgagctagagtcaacaccaaggcccagggggaatggagtgaagatctcactgcttggacccttagtgacattcttcctcctcaaccagaaaacatcaagatttccaacattacacactcctcagctgtgatttcttggacaatattggatggctattctatttcttctattactatccgttacaaggttcaaggcaagaatgaagaccagcacgttgatgtgaagataaagaatgccaccatcactcagtatcagctcaagggcctagagcctgaaacagcataccaggtggacatttttgcagagaacaacatagggtcaagcaacccagccttttctcatgaactggtgaccctcccagaatctcaagcaccagcggacctcggaggggggaagatgctgcttatagccatccttggctctgctggaatgacctgcctgactgtgctgttggcctttctgatcatattgcaattgaagagggcaaatgtgcaaaggagaatggcccaagccttccaaaacgtgagggaagaaccagctgtgcagttcaactcagggactctggccctaaacaggaaggtcaaaaacaacccagatcctacaatttatccagtgcttgactggaatgacatcaaatttcaagatgtgattggggagggcaattttggccaagttcttaaggcgcgcatcaagaaggatgggttacggatggatgctgccatcaaaagaatgaaagaatatgcctccaaagatgatcacagggactttgcaggagaactggaagttctttgtaaacttggacaccatccaaacatcatcaatctcttaggagcatgtgaacatcgaggctacttgtacctggccattgagtacgcgccccatggaaaccttctggacttccttcgcaagagccgtgtgctggagacggacccagcatttgccattgccaatagcaccgcgtccacactgtcctcccagcagctccttcacttcgctgccgacgtggcccggggcatggactacttgagccaaaaacagtttatccacagggatctggctgccagaaacattttagttggtgaaaactatgtggcaaaaatagcagattttggattgtcccgaggtcaagaggtgtatgtgaaaaagacaatgggaaggctcccagtgcgctggatggccatcgagtcactgaattacagtgtgtacacaaccaacagtgatgtatggtcctatggtgtgttactatgggagattgttagcttaggaggcacaccctactgcgggatgacttgtgcagaactctacgagaagctgccccagggctacagactggagaagcccctgaactgtgatgatgaggtgtatgatctaatgagacaatgctggcgggagaagccttatgagaggccatcatttgcccagatattggtgtccttaaacagaatgttagaggagcgaaagacctacgtgaataccacgctttatgagaagtttacttatgcaggaattgactgttctgctgaagaagcggcctag

SEQ ID NO: 102 - protein, 1124 aa, Homo sapiens
MDSLASLVLCGVSLLLSGTVEGAMDLILINSLPLVSDAETSLTCIASGWRPHEPITIGRDFEALMNQHQDPLEVTQDVTREWAKKVVWKREKASKINGAYFCEGRVRGEAIRIRTMKMRQQASFLPATLTMTVDKGDNVNISFKKVLIKEEDAVIYKNGSFIHSVPRHEVPDILEVHLPHAQPQDAGVYSARYIGGNLFTSAFTRLIVRRCEAQKWGPECNHLCTACMNNGVCHEDTGECICPPGFMGRTCEKACELHTFGRTCKERCSGQEGCKSYVFCLPDPYGCSCATGWKGLQCNEACHPGFYGPDCKLRCSCNNGEMCDRFQGCLCSPGWQGLQCEREGIPRMTPKIVDLPDHIEVNSGKFNPICKASGWPLPTNEEMTLVKPDGTVLHPKDFNHTDHFSVAIFTIHRILPPDSGVWVCSVNTVAGMVEKPFNISVKVLPKPLNAPNVIDTGHNFAVINISSEPYFGDGPIKSKKLLYKPVNHYEAWQHIQVTNEIVTLNYLEPRTEYELCVQLVRRGEGGEGHPGPVRRFTTASIGLPPPRGLNLLPKSQTTLNLTWQPIFPSSEDDFYVEVERRSVQKSDQQNIKVPGNLTSVLLNNLHPREQYVVRARVNTKAQGEWSEDLTAWTLSDILPPQPENIKISNITHSSAVISWTILDGYSISSITIRYKVQGKNEDQHVDVKIKNATITQYQLKGLEPETAYQVDIFAENNIGSSNPAFSHELVTLPESQAPADLGGGKMLLIAILGSAGMTCLTVLLAFLIILQLKRANVQRRMAQAFQNVREEPAVQFNSGTLALNRKVKNNPDPTIYPVLDWNDIKFQDVIGEGNFGQVLKARIKKDGLRMDAAIKRMKEYASKDDHRDFAGELEVLCKLGHHPNIINLLGACEHRGYLYLAIEYAPHGNLLDFLRKSRVLETDPAFAIANSTASTLSSQQLLHFAADVARGMDYLSQKQFIHRDLAARNILVGENYVAKIADFGLSRGQEVYVKKTMGRLPVRWMAIESLNYSVYTTNSDVWSYGVLLWEIVSLGGTPYCGMTCAELYEKLPQGYRLEKPLNCDDEVYDLMRQCWREKPYERPSFAQILVSLNRMLEERKTYVNTTLYEKFTYAGIDCSAEEAA

SEQ ID NO: 103 - DNA, 3375 bp, Homo sapiens
  CDS (1)..(3375)
atggactctttagccagcttagttctctgtggagtcagcttgctcctttctggaactgtggaaggtgccatggacttgatcttgatcaattccctacctcttgtatctgatgctgaaacatctctcacctgcattgcctctgggtggcgcccccatgagcccatcaccataggaagggactttgaagccttaatgaaccagcaccaggatccgctggaagttactcaagatgtgaccagagaatgggctaaaaaagttgtttggaagagagaaaaggctagtaagatcaatggtgcttatttctgtgaagggcgagttcgaggagaggcaatcaggatacgaaccatgaagatgcgtcaacaagcttccttcctaccagctactttaactatgactgtggacaagggagataacgtgaacatatctttcaaaaaggtattgattaaagaagaagatgcagtgatttacaaaaatggttccttcatccattcagtgccccggcatgaagtacctgatattctagaagtacacctgcctcatgctcagccccaggatgctggagtgtactcggccaggtatataggaggaaacctcttcacctcggccttcaccaggctgatagtccggagatgtgaagcccagaagtggggacctgaatgcaaccatctctgtactgcttgtatgaacaatggtgtctgccatgaagatactggagaatgcatttgccctcctgggtttatgggaaggacgtgtgagaaggcttgtgaactgcacacgtttggcagaacttgtaaagaaaggtgcagtggacaagagggatgcaagtcttatgtgttctgtctccctgacccctatgggtgttcctgtgccacaggctggaagggtctgcagtgcaatgaagcatgccaccctggtttttacgggccagattgtaagcttaggtgcagctgcaacaatggggagatgtgtgatcgcttccaaggatgtctctgctctccaggatggcaggggctccagtgtgagagagaaggcataccgaggatgaccccaaagatagtggatttgccagatcatatagaagtaaacagtggtaaatttaatcccatttgcaaagcttctggctggccgctacctactaatgaagaaatgaccctggtgaagccggatgggacagtgctccatccaaaagactttaaccatacggatcatttctcagtagccatattcaccatccaccggatcctcccccctgactcaggagtttgggtctgcagtgtgaacacagtggctgggatggtggaaaagcccttcaacatttctgttaaagttcttccaaagcccctgaatgccccaaacgtgattgacactggacataactttgctgtcatcaacatcagctctgagccttactttggggatggaccaatcaaatccaagaagcttctatacaaacccgttaatcactatgaggcttggcaacatattcaagtgacaaatgagattgttacactcaactatttggaacctcggacagaatatgaactctgtgtgcaactggtccgtcgtggagagggtggggaagggcatcctggacctgtgagacgcttcacaacagcttctatcggactccctcctccaagaggtctaaatctcctgcctaaaagtcagaccactctaaatttgacctggcaaccaatatttccaagctcggaagatgacttttatgttgaagtggagagaaggtctgtgcaaaaaagtgatcagcagaatattaaagttccaggcaacttgacttcggtgctacttaacaacttacatcccagggagcagtacgtggtccgagctagagtcaacaccaaggcccagggggaatggagtgaagatctcactgcttggacccttagtgacattcttcctcctcaaccagaaaacatcaagatttccaacattacacactcctcagctgtgatttcttggacaatattggatggctattctatttcttctattactatccgttacaaggttcaaggcaagaatgaagaccagcacgttgatgtgaagataaagaatgccaccatcactcagtatcagctcaagggcctagagcctgaaacagcataccaggtggacatttttgcagagaacaacatagggtcaagcaacccagccttttctcatgaactggtgaccctcccagaatctcaagcaccagcggacctcggaggggggaagatgctgcttatagccatccttggctctgctggaatgacctgcctgactgtgctgttggcctttctgatcatattgcaattgaagagggcaaatgtgcaaaggagaatggcccaagccttccaaaacgtgagggaagaaccagctgtgcagttcaactcagggactctggccctaaacaggaaggtcaaaaacaacccagatcctacaatttatccagtgcttgactggaatgacatcaaatttcaagatgtgattggggagggcaattttggccaagttcttaaggcgcgcatcaagaaggatgggttatggatggatgctgccatcaaaagaatgaaagaatatgcctccaaagatgatcacagggactttgcaggagaactggaagttctttgtaaacttggacaccatccaaacatcatcaatctcttaggagcatgtgaacatcgaggctacttgtacctggccattgagtacgcgccccatggaaaccttctggacttccttcgcaagagccgtgtgctggagacggacccagcatttgccattgccaatagcaccgcgtccacactgtcctcccagcagctccttcacttcgctgccgacgtggcccggggcatggactacttgagccaaaaacagtttatccacagggatctggctgccagaaacattttagttggtgaaaactatgtggcaaaaatagcagattttggattgtcccgaggtcaagaggtgtatgtgaaaaagacaatgggaaggctcccagtgcgctggatggccatcgagtcactgaattacagtgtgtacacaaccaacagtgatgtatggtcctatggtgtgttactatgggagattgttagcttaggaggcacaccctactgcgggatgacttgtgcagaactctacgagaagctgccccagggctacagactggagaagcccctgaactgtgatgatgaggtgtatgatctaatgagacaatgctggcgggagaagccttatgagaggccatcatttgcccagatattggtgtccttaaacagaatgttagaggagcgaaagacctacgtgaataccacgctttatgagaagtttacttatgcaggaattgactgttctgctgaagaagcggcctag

SEQ ID NO: 104 - protein, 1124 aa, Homo sapiens
MDSLASLVLCGVSLLLSGTVEGAMDLILINSLPLVSDAETSLTCIASGWRPHEPITIGRDFEALMNQHQDPLEVTQDVTREWAKKVVWKREKASKINGAYFCEGRVRGEAIRIRTMKMRQQASFLPATLTMTVDKGDNVNISFKKVLIKEEDAVIYKNGSFIHSVPRHEVPDILEVHLPHAQPQDAGVYSARYIGGNLFTSAFTRLIVRRCEAQKWGPECNHLCTACMNNGVCHEDTGECICPPGFMGRTCEKACELHTFGRTCKERCSGQEGCKSYVFCLPDPYGCSCATGWKGLQCNEACHPGFYGPDCKLRCSCNNGEMCDRFQGCLCSPGWQGLQCEREGIPRMTPKIVDLPDHIEVNSGKFNPICKASGWPLPTNEEMTLVKPDGTVLHPKDFNHTDHFSVAIFTIHRILPPDSGVWVCSVNTVAGMVEKPFNISVKVLPKPLNAPNVIDTGHNFAVINISSEPYFGDGPIKSKKLLYKPVNHYEAWQHIQVTNEIVTLNYLEPRTEYELCVQLVRRGEGGEGHPGPVRRFTTASIGLPPPRGLNLLPKSQTTLNLTWQPIFPSSEDDFYVEVERRSVQKSDQQNIKVPGNLTSVLLNNLHPREQYVVRARVNTKAQGEWSEDLTAWTLSDILPPQPENIKISNITHSSAVISWTILDGYSISSITIRYKVQGKNEDQHVDVKIKNATITQYQLKGLEPETAYQVDIFAENNIGSSNPAFSHELVTLPESQAPADLGGGKMLLIAILGSAGMTCLTVLLAFLIILQLKRANVQRRMAQAFQNVREEPAVQFNSGTLALNRKVKNNPDPTIYPVLDWNDIKFQDVIGEGNFGQVLKARIKKDGLWMDAAIKRMKEYASKDDHRDFAGELEVLCKLGHHPNIINLLGACEHRGYLYLAIEYAPHGNLLDFLRKSRVLETDPAFAIANSTASTLSSQQLLHFAADVARGMDYLSQKQFIHRDLAARNILVGENYVAKIADFGLSRGQEVYVKKTMGRLPVRWMAIESLNYSVYTTNSDVWSYGVLLWEIVSLGGTPYCGMTCAELYEKLPQGYRLEKPLNCDDEVYDLMRQCWREKPYERPSFAQILVSLNRMLEERKTYVNTTLYEKFTYAGIDCSAEEAA

SEQ ID NO: 105 - DNA, 814 bp, Artificial Sequence
  Synthetic
gaggaaccgagaggctgagactaacccagaaacatccaattctcaaactgaagctcgcactctcgcctccagcatgaactccttctccacaagcgccttcggtccagttgccttctccctgggcctgctcctggtgttgcctgctgccttccctgccccagtcttcacactcgaagatttcgttggggactggcgacagacagccggctacaacctggaccaagtccttgaacagggaggtgtgtccagtttgtttcagaatctcggggtgtccgtaactccgatccaaaggattgtcctgagcggtgaaaatgggctgaagatcgacatccatgtcatcatcccgtatgaaggtctgagcggcgaccaaatgggccagatcgaaaaaatttttaaggtggtgtaccctgtggatgatcatcactttaaggtgatcctgcactatggcacactggtaatcgacggggttacgccgaacatgatcgactatttcggacggccgtatgaaggcatcgccgtgttcgacggcaaaaagatcactgtaacagggaccctgtggaacggcaacaaaattatcgacgagcgcctgatcaaccccgacggctccctgctgttccgagtaaccatcaacggagtgaccggctggcggctgtgcgaacgcattctggcgtaaggctgctgcagctgcatgggtgcctgctgctgcctgccttggcctgatggccaggccagagtgctgccagtcctctgcatgttctgctcttgtgcccttctgagcccacaataaaggctgagctcttatcttgcaaaaggc

SEQ ID NO: 106 - DNA, 984 bp, Artificial Sequence
  Synthetic
ataaaagcccaggggcaagcggtccggataacggctagcctgaggagctgctgcgacagtccactacctttttcgagagtgactcccgttgtcccaaggcttcccagagcgaacctgtgcggctgcaggcaccggcgcgtcgagtttccggcgtccggaaggaccgagctcttctcgcgaatccagtgttccgtttccagcccccaatctcagagcggagccgacagagagcagggaaccggcatgaactccttctccacaagcgccttcggtccagttgccttctccctgggcctgctcctggtgttgcctgctgccttccctgccccagtcttcacactcgaagatttcgttggggactggcgacagacagccggctacaacctggaccaagtccttgaacagggaggtgtgtccagtttgtttcagaatctcggggtgtccgtaactccgatccaaaggattgtcctgagcggtgaaaatgggctgaagatcgacatccatgtcatcatcccgtatgaaggtctgagcggcgaccaaatgggccagatcgaaaaaatttttaaggtggtgtaccctgtggatgatcatcactttaaggtgatcctgcactatggcacactggtaatcgacggggttacgccgaacatgatcgactatttcggacggccgtatgaaggcatcgccgtgttcgacggcaaaaagatcactgtaacagggaccctgtggaacggcaacaaaattatcgacgagcgcctgatcaaccccgacggctccctgctgttccgagtaaccatcaacggagtgaccggctggcggctgtgcgaacgcattctggcgtaaggctgctgcagctgcatgggtgcctgctgctgcctgccttggcctgatggccaggccagagtgctgccagtcctctgcatgttctgctcttgtgcccttctgagcccacaataaaggctgagctcttatcttgcaaaaggc

SEQ ID NO: 107 - DNA, 1735 bp, Artificial Sequence
  Synthetic
gaggaaccgagaggctgagactaacccagaaacatccaattctcaaactgaagctcgcactctcgcctccagcatgaaagtctctgccgcccttctgtgcctgctgctcatagcagccaccttcattccccaagggctcgctcacatagggtgcagcaatcagcgccgaagtccagaaaacagtgggagaagatataaccggattcaacatgggcaatgtgcctacactttcattcttccagaacacgatggcaactgtcgtgagagtacgacagaccagtacaacacaaacgctctgcagagagatgctccacacgtggaaccggatttctcttcccagaaacttcaacatctggaacatgtgatggaaaattatactcagtggctgcaaaaacttgagaattacattgtggaaaacatgaagtcggagatggcccagatacagcagaatgcagttcagaaccacacggctaccatgctggagataggaaccagcctcctctctcagactgcagagcagaccagaaagctgacagatgttgagacccaggtactaaatcaaacttctcgacttgagatacagctgctggagaattcattatccacctacaagctagagaagcaacttcttcaacagacaaatgaaatcttgaagatccatgaaaaaaacagtttattagaacataaaatcttagaaatggaaggaaaacacaaggaagagttggacaccttaaaggaagagaaagagaaccttcaaggcttggttactcgtcaaacatatataatccaggagctggaaaagcaattaaacagagctaccaccaacaacagtgtccttcagaagcagcaactggagctgatggacacagtccacaaccttgtcaatctttgcactaaagaaggtgttttactaaagggaggaaaaagagaggaagagaaaccatttagagactgtgcagatgtatatcaagctggttttaataaaagtggaatctacactatttatattaataatatgccagaacccaaaaaggtgttttgcaatatggatgtcaatgggggaggttggactgtaatacaacatcgtgaagatggaagtctagatttccaaagaggctggaaggaatataaaatgggttttggaaatccctccggtgaatattggctggggaatgagtttatttttgccattaccagtcagaggcagtacatgctaagaattgagttaatggactgggaagggaaccgagcctattcacagtatgacagattccacataggaaatgaaaagcaaaactataggttgtatttaaaaggtcacactgggacagcaggaaaacagagcagcctgatcttacacggtgctgatttcagcactaaagatgctgataatgacaactgtatgtgcaaatgtgccctcatgttaacaggaggatggtggtttgatgcttgtggcccctccaatctaaatggaatgttctatactgcgggacaaaaccatggaaaactgaatgggataaagtggcactacttcaaagggcccagttactccttacgttccacaactatgatgattcgacctttagatttttgaggctgctgcagctgcatgggtgcctgctgctgcctgccttggcctgatggccaggccagagtgctgccagtcctctgcatgttctgctcttgtgcccttctgagcccacaataaaggctgagctcttatcttgcaaaaggc

SEQ ID NO: 108 - DNA, 1150 bp, Artificial Sequence
  Synthetic
gaggaaccgagaggctgagactaacccagaaacatccaattctcaaactgaagctcgcactctcgcctccagcatgaaagtctctgccgcccttctgtgcctgctgctcatagcagccaccttcattccccaagggctcgctgggatcttagacttgggcccgcagatgcttcgggaactgcaggaaaccaacgcggcgctgcaggacgtgcgggagctgctgcggcagcaggtcagggagatcacgttcctgaaaaacacggtgatggagtgtgacgcgtgcggaggctcccttgtcaatctttgcactaaagaaggtgttttactaaagggaggaaaaagagaggaagagaaaccatttagagactgtgcagatgtatatcaagctggttttaataaaagtggaatctacactatttatattaataatatgccagaacccaaaaaggtgttttgcaatatggatgtcaatgggggaggttggactgtaatacaacatcgtgaagatggaagtctagatttccaaagaggctggaaggaatataaaatgggttttggaaatccctccggtgaatattggctggggaatgagtttatttttgccattaccagtcagaggcagtacatgctaagaattgagttaatggactgggaagggaaccgagcctattcacagtatgacagattccacataggaaatgaaaagcaaaactataggttgtatttaaaaggtcacactgggacagcaggaaaacagagcagcctgatcttacacggtgctgatttcagcactaaagatgctgataatgacaactgtatgtgcaaatgtgccctcatgttaacaggaggatggtggtttgatgcttgtggcccctccaatctaaatggaatgttctatactgcgggacaaaaccatggaaaactgaatgggataaagtggcactacttcaaagggcccagttactccttacgttccacaactatgatgattcgacctttagatttttgaggctgctgcagctgcatgggtgcctgctgctgcctgccttggcctgatggccaggccagagtgctgccagtcctctgcatgttctgctcttgtgcccttctgagcccacaataaaggctgagctcttatcttgcaaaaggc

SEQ ID NO: 109 - DNA, 817 bp, Artificial Sequence
  Synthetic
catatcttcattcttcactctttccccccccccccttatcctcctatctaatcctctcatctctctcctcctcttcctccaacaacaactaacaatgaaagtctctgccgcccttctgtgcctgctgctcatagcagccaccttcattccccaagggctcgctgtcttcacactcgaagatttcgttggggactggcgacagacagccggctacaacctggaccaagtccttgaacagggaggtgtgtccagtttgtttcagaatctcggggtgtccgtaactccgatccaaaggattgtcctgagcggtgaaaatgggctgaagatcgacatccatgtcatcatcccgtatgaaggtctgagcggcgaccaaatgggccagatcgaaaaaatttttaaggtggtgtaccctgtggatgatcatcactttaaggtgatcctgcactatggcacactggtaatcgacggggttacgccgaacatgatcgactatttcggacggccgtatgaaggcatcgccgtgttcgacggcaaaaagatcactgtaacagggaccctgtggaacggcaacaaaattatcgacgagcgcctgatcaaccccgacggctccctgctgttccgagtaaccatcaacggagtgaccggctggcggctgtgcgaacgcattctggcgtaaggctgctgcagctgcatgggtgcctgctgctgcctgccttggcctgatggccaggccagagtgctgccagtcctctgcatgttctgctcttgtgcccttctgagcccacaataaaggctgagctcttatcttgcaaaaggc

SEQ ID NO: 110 - DNA, 978 bp, Artificial Sequence
  Synthetic
gtggcagctcacagctattgtggtgggaaagggagggtggttggtggatgtcacagcttgggctttatctcccccagcagtggggactccacagcccctgggctacataacagcaagacagtccggagctgtagcagacctgattgagcctttgcagcagctgagagcatggcctagggtgggcggcaccattgtccagcagctgagtttcccagggaccttggagatagccgcagccctcatttgcaggggaagatgaaagtctctgccgcccttctgtgcctgctgctcatagcagccaccttcattccccaagggctcgctgtcttcacactcgaagatttcgttggggactggcgacagacagccggctacaacctggaccaagtccttgaacagggaggtgtgtccagtttgtttcagaatctcggggtgtccgtaactccgatccaaaggattgtcctgagcggtgaaaatgggctgaagatcgacatccatgtcatcatcccgtatgaaggtctgagcggcgaccaaatgggccagatcgaaaaaatttttaaggtggtgtaccctgtggatgatcatcactttaaggtgatcctgcactatggcacactggtaatcgacggggttacgccgaacatgatcgactatttcggacggccgtatgaaggcatcgccgtgttcgacggcaaaaagatcactgtaacagggaccctgtggaacggcaacaaaattatcgacgagcgcctgatcaaccccgacggctccctgctgttccgagtaaccatcaacggagtgaccggctggcggctgtgcgaacgcattctggcgtaaggctgctgcagctgcatgggtgcctgctgctgcctgccttggcctgatggccaggccagagtgctgccagtcctctgcatgttctgctcttgtgcccttctgagcccacaataaaggctgagctcttatcttgcaaaaggc

SEQ ID NO: 111 - DNA, 975 bp, Artificial Sequence; identical to SEQ ID NO: 82
  Synthetic

SEQ ID NO: 112 - DNA, 778 bp, Artificial Sequence
  Synthetic
gggaaataagagagaaaagaagagtaagaagaaatataagaccccggcgccgccaccatgaaagtctctgccgcccttctgtgcctgctgctcatagcagccaccttcattccccaagggctcgctgtcttcacactcgaagatttcgttggggactggcgacagacagccggctacaacctggaccaagtccttgaacagggaggtgtgtccagtttgtttcagaatctcggggtgtccgtaactccgatccaaaggattgtcctgagcggtgaaaatgggctgaagatcgacatccatgtcatcatcccgtatgaaggtctgagcggcgaccaaatgggccagatcgaaaaaatttttaaggtggtgtaccctgtggatgatcatcactttaaggtgatcctgcactatggcacactggtaatcgacggggttacgccgaacatgatcgactatttcggacggccgtatgaaggcatcgccgtgttcgacggcaaaaagatcactgtaacagggaccctgtggaacggcaacaaaattatcgacgagcgcctgatcaaccccgacggctccctgctgttccgagtaaccatcaacggagtgaccggctggcggctgtgcgaacgcattctggcgtaataataggctggagcctcggtggcctagcttcttgccccttgggcctccccccagcccctcctccccttcctgcacccgtaccccctccataaagtaggaaacactacagtggtctttgaataaagtctgagtgggcggc

SEQ ID NO: 113 - DNA, 796 bp, Artificial Sequence
  Synthetic
gaggaaccgagaggctgagactaacccagaaacatccaattctcaaactgaagctcgcactctcgccgccaccatgaaagtctctgccgcccttctgtgcctgctgctcatagcagccaccttcattccccaagggctcgctgtcttcacactcgaagatttcgttggggactggcgacagacagccggctacaacctggaccaagtccttgaacagggaggtgtgtccagtttgtttcagaatctcggggtgtccgtaactccgatccaaaggattgtcctgagcggtgaaaatgggctgaagatcgacatccatgtcatcatcccgtatgaaggtctgagcggcgaccaaatgggccagatcgaaaaaatttttaaggtggtgtaccctgtggatgatcatcactttaaggtgatcctgcactatggcacactggtaatcgacggggttacgccgaacatgatcgactatttcggacggccgtatgaaggcatcgccgtgttcgacggcaaaaagatcactgtaacagggaccctgtggaacggcaacaaaattatcgacgagcgcctgatcaaccccgacggctccctgctgttccgagtaaccatcaacggagtgaccggctggcggctgtgcgaacgcattctggcgtaaggctgctgcagctgcatgggtgcctgctgctgcctgccttggcctgatggccaggccagagtgctgccagtcctctgcatgttctgctcttgtgcccttctgagcccacaataaaggctgagctcttatcttgcaaaaggc

SEQ ID NO: 114 - DNA, 1144 bp, Artificial Sequence
  Synthetic
gaggaaccgagaggctgagactaacccagaaacatccaattctcaaactgaagctcgcactctcgcctccagcatgaaagtctctgccgcccttctgtgcctgctgctcatagcagccaccttcattccccaagggctcgctgggatcttagaggaagacccggccgcctgcgagtccctggtgaaattccaagccaaagtggaggggctgctgcaggccctgaccaggaaactggaagctgtgagtaagcggctggccatcctggagaacacagttgtcggctcccttgtcaatcttgccactaaagaaggtgttttactaaagggaggaaaaagagaggaagagaaaccatttagagactgtgcagatgtatatcaagctggttttaataaaagtggaatctacactatttatattaataatatgccagaacccaaaaaggtgttttgcaatatggatgtcaatgggggaggttggactgtaatacaacatcgtgaagatggaagtctagatttccaaagaggctggaaggaatataaaatgggttttggaaatccctccggtgaatattggctggggaatgagtttatttttgccattaccagtcagaggcagtacatgctaagaattgagttaatggactgggaagggaaccgagcctattcacagtatgacagattccacataggaaatgaaaagcaaaactataggttgtatttaaaaggtcacactgggacagcaggaaaacagagcagcctgatcttacacggtgctgatttcagcactaaagatgctgataatgacaactgtatgtgcaaatgtgccctcatgttaacaggaggatggtggtttgatgcttgtggcccctccaatctaaatggaatgttctatactgcgggacaaaaccatggaaaactgaatgggataaagtggcactacttcaaagggcccagttactccttacgttccacaactatgatgattcgacctttagatttttgaggctgctgcagctgcatgggtgcctgctgctgcctgccttggcctgatggccaggccagagtgctgccagtcctctgcatgttctgctcttgtgcccttctgagcccacaataaaggctgagctcttatcttgcaaaaggc

SEQ ID NO: 115 - DNA, 3589 bp, Artificial Sequence
  Synthetic
gaggaaccgagaggctgagactaacccagaaacatccaattctcaaactgaagctcgcactctcgcctccagcatggactctttagccagcttagttctctgtggagtcagcttgctcctttctggaactgtggaaggtgccatggacttgatcttgatcaattccctacctcttgtatctgatgctgaaacatctctcacctgcattgcctctgggtggcgcccccatgagcccatcaccataggaagggactttgaagccttaatgaaccagcaccaggacccgctggaagttactcaagatgtgaccagagaatgggctaaaaaagttgtttggaagagagaaaaggctagtaagatcaatggtgcttatttctgtgaagggcgagttcgaggagaggcaatcaggatacgaaccatgaagatgcgtcaacaagcttccttcctaccagctactttaactatgactgtggacaagggagataacgtgaacatatctttcaaaaaggtattgattaaagaagaagatgcagtgatttacaaaaatggttccttcatccattcagtgccccggcatgaagtacctgatattctagaagtacacctgcctcatgctcagccccaggatgctggagtgtactcggccaggtatataggaggaaacctcttcacctcggccttcaccaggctgatagtccggagatgtgaagcccagaagtggggacctgaatgcaaccatctctgtactgcttgtatgaacaatggtgtctgccatgaagatactggagaatgcatttgccctcctgggtttatgggaaggacgtgtgagaaggcttgtgaactgcacacgtttggcagaacttgtaaagaaaggtgcagtggacaagagggatgcaagtcttatgtgttctgtctccctgacccctatgggtgttcctgtgccacaggctggaagggtctgcagtgcaatgaagcatgccaccctggtttttacgggccagattgtaagcttaggtgcagctgcaacaatggggagatgtgtgatcgcttccaaggatgtctctgctctccaggatggcaggggctccagtgtgagagagaaggcataccgaggatgaccccaaagatagtggatttgccagatcatatagaagtaaacagtggtaaatttaatcccatttgcaaagcttctggctggccgctacctactaatgaagaaatgaccctggtgaagccggatgggacagtgctccatccaaaagactttaaccatacggatcatttctcagtagccatattcaccatccacagaatcctcccccctgactcaggagtttgggtctgcagtgtgaacacagtggctgggatggtggaaaagcccttcaacatttctgttaaagttcttccaaagcccctgaatgccccaaacgtgattgacactggacataactttgctgtcatcaacatcagctctgagccttactttggggatggaccaatcaaatccaagaagcttctatacaaacccgttaatcactatgaggcttggcaacatattcaagtgacaaatgagattgttacactcaactatttggaacctcggacagaatatgaactctgtgtgcaactggtccgtcgtggagagggtggggaagggcatcctggacctgtgagacgcttcacaacagcttctatcggactccctcctccaagaggtctaaatctcctgcctaaaagtcagaccactctaaatttgacctggcaaccaatatttccaagctcggaagatgacttttatgttgaagtggagagaaggtctgtgcaaaaaagtgatcagcagaatattaaagttccaggcaacttgacttcggtgctacttaacaacttacatcccagggagcagtacgtggtccgagctagagtcaacaccaaggcccagggggaatggagtgaagatctcactgcttggacccttagtgacattcttcctcctcaaccagaaaacatcaagatttccaacattacacactcctcagctgtgatttcttggacaatattggatggctattctatttcttctattactatccgttacaaggttcaaggcaagaatgaagaccagcacgttgatgtgaagataaagaatgccaccatcactcagtatcagctcaagggcctagagcctgaaacagcataccaggtggacatttttgcagagaacaacatagggtcaagcaacccagccttttctcatgaactggtgaccctcccagaatctcaagcaccagcggacctcggaggggggaagatgctgcttatagccatccttggctctgctggaatgacctgcctgactgtgctgttggcctttctgatcatattgcaattgaagagggcaaatgtgcaaaggagaatggcccaagccttccaaaacgtgagggaagaaccagctgtgcagttcaactcagggactctggccctaaacaggaaggtcaaaaacaacccagatcctacaatttatccagtgcttgactggaatgacatcaaatttcaagatgtgattggggagggcaattttggccaagttcttaaggcgcgcatcaagaaggatgggttacggatggatgctgccatcaaaagaatgaaagaatatgcctccaaagatgatcacagggactttgcaggagaactggaagttctttgtaaacttggacaccatccaaacatcatcaatctcttaggagcatgtgaacatcgaggctacttgtacctggccattgagtacgcgccccatggaaaccttctggacttccttcgcaagagccgtgtgctggagacggacccagcatttgccattgccaatagcaccgcgtccacactgtcctcccagcagctccttcacttcgctgccgacgtggcccggggcatggactacttgagccaaaaacagtttatccacagggatctggctgccagaaacattttagttggtgaaaactatgtggcaaaaatagcagattttggattgtcccgaggtcaagaggtgtatgtgaaaaagacaatgggaaggctcccagtgcgctggatggccatcgagtcactgaattacagtgtgtacacaaccaacagtgatgtatggtcctatggtgtgttactatgggagattgttagcttaggaggcacaccctactgcgggatgacttgtgcagaactctacgagaagctgccccagggctacagactggagaagcccctgaactgtgatgatgaggtgtatgatctaatgagacaatgctggcgggagaagccttatgagaggccatcatttgcccagatattggtgtccttaaacagaatgttagaggagcgaaagacctacgtgaataccacgctttatgagaagtttacttatgcaggaattgactgttctgctgaagaagcggcctagggctgctgcagctgcatgggtgcctgctgctgcctgccttggcctgatggccaggccagagtgctgccagtcctctgcatgttctgctcttgtgcccttctgagcccacaataaaggctgagctcttatcttgcaaaaggc

SEQ ID NO: 116 - DNA, 3589 bp, Artificial Sequence
  Synthetic
gaggaaccgagaggctgagactaacccagaaacatccaattctcaaactgaagctcgcactctcgcctccagcatggactctttagccagcttagttctctgtggagtcagcttgctcctttctggaactgtggaaggtgccatggacttgatcttgatcaattccctacctcttgtatctgatgctgaaacatctctcacctgcattgcctctgggtggcgcccccatgagcccatcaccataggaagggactttgaagccttaatgaaccagcaccaggacccgctggaagttactcaagatgtgaccagagaatgggctaaaaaagttgtttggaagagagaaaaggctagtaagatcaatggtgcttatttctgtgaagggcgagttcgaggagaggcaatcaggatacgaaccatgaagatgcgtcaacaagcttccttcctaccagctactttaactatgactgtggacaagggagataacgtgaacatatctttcaaaaaggtattgattaaagaagaagatgcagtgatttacaaaaatggttccttcatccattcagtgccccggcatgaagtacctgatattctagaagtacacctgcctcatgctcagccccaggatgctggagtgtactcggccaggtatataggaggaaacctcttcacctcggccttcaccaggctgatagtccggagatgtgaagcccagaagtggggacctgaatgcaaccatctctgtactgcttgtatgaacaatggtgtctgccatgaagatactggagaatgcatttgccctcctgggtttatgggaaggacgtgtgagaaggcttgtgaactgcacacgtttggcagaacttgtaaagaaaggtgcagtggacaagagggatgcaagtcttatgtgttctgtctccctgacccctatgggtgttcctgtgccacaggctggaagggtctgcagtgcaatgaagcatgccaccctggtttttacgggccagattgtaagcttaggtgcagctgcaacaatggggagatgtgtgatcgcttccaaggatgtctctgctctccaggatggcaggggctccagtgtgagagagaaggcataccgaggatgaccccaaagatagtggatttgccagatcatatagaagtaaacagtggtaaatttaatcccatttgcaaagcttctggctggccgctacctactaatgaagaaatgaccctggtgaagccggatgggacagtgctccatccaaaagactttaaccatacggatcatttctcagtagccatattcaccatccacagaatcctcccccctgactcaggagtttgggtctgcagtgtgaacacagtggctgggatggtggaaaagcccttcaacatttctgttaaagttcttccaaagcccctgaatgccccaaacgtgattgacactggacataactttgctgtcatcaacatcagctctgagccttactttggggatggaccaatcaaatccaagaagcttctatacaaacccgttaatcactatgaggcttggcaacatattcaagtgacaaatgagattgttacactcaactatttggaacctcggacagaatatgaactctgtgtgcaactggtccgtcgtggagagggtggggaagggcatcctggacctgtgagacgcttcacaacagcttctatcggactccctcctccaagaggtctaaatctcctgcctaaaagtcagaccactctaaatttgacctggcaaccaatatttccaagctcggaagatgacttttatgttgaagtggagagaaggtctgtgcaaaaaagtgatcagcagaatattaaagttccaggcaacttgacttcggtgctacttaacaacttacatcccagggagcagtacgtggtccgagctagagtcaacaccaaggcccagggggaatggagtgaagatctcactgcttggacccttagtgacattcttcctcctcaaccagaaaacatcaagatttccaacattacacactcctcagctgtgatttcttggacaatattggatggctattctatttcttctattactatccgttacaaggttcaaggcaagaatgaagaccagcacgttgatgtgaagataaagaatgccaccatcactcagtatcagctcaagggcctagagcctgaaacagcataccaggtggacatttttgcagagaacaacatagggtcaagcaacccagccttttctcatgaactggtgaccctcccagaatctcaagcaccagcggacctcggaggggggaagatgctgcttatagccatccttggctctgctggaatgacctgcctgactgtgctgttggcctttctgatcatattgcaattgaagagggcaaatgtgcaaaggagaatggcccaagccttccaaaacgtgagggaagaaccagctgtgcagttcaactcagggactctggccctaaacaggaaggtcaaaaacaacccagatcctacaatttatccagtgcttgactggaatgacatcaaatttcaagatgtgattggggagggcaattttggccaagttcttaaggcgcgcatcaagaaggatgggttatggatggatgctgccatcaaaagaatgaaagaatatgcctccaaagatgatcacagggactttgcaggagaactggaagttctttgtaaacttggacaccatccaaacatcatcaatctcttaggagcatgtgaacatcgaggctacttgtacctggccattgagtacgcgccccatggaaaccttctggacttccttcgcaagagccgtgtgctggagacggacccagcatttgccattgccaatagcaccgcgtccacactgtcctcccagcagctccttcacttcgctgccgacgtggcccggggcatggactacttgagccaaaaacagtttatccacagggatctggctgccagaaacattttagttggtgaaaactatgtggcaaaaatagcagattttggattgtcccgaggtcaagaggtgtatgtgaaaaagacaatgggaaggctcccagtgcgctggatggccatcgagtcactgaattacagtgtgtacacaaccaacagtgatgtatggtcctatggtgtgttactatgggagattgttagcttaggaggcacaccctactgcgggatgacttgtgcagaactctacgagaagctgccccagggctacagactggagaagcccctgaactgtgatgatgaggtgtatgatctaatgagacaatgctggcgggagaagccttatgagaggccatcatttgcccagatattggtgtccttaaacagaatgttagaggagcgaaagacctacgtgaataccacgctttatgagaagtttacttatgcaggaattgactgttctgctgaagaagcggcctagggctgctgcagctgcatgggtgcctgctgctgcctgccttggcctgatggccaggccagagtgctgccagtcctctgcatgttctgctcttgtgcccttctgagcccacaataaaggctgagctcttatcttgcaaaaggc

SEQ ID NO: 117 - DNA, 3207 bp, Homo sapiens
  CDS (1)..(3207)
atgcctccacgaccatcatcaggtgaactgtggggcatccacttgatgcccccaagaatcctagtagaatgtttactaccaaatggaatgatagtgactttagaatgcctccgtgaggctacattaataaccataaagcatgaactatttaaagaagcaagaaaataccccctccatcaacttcttcaagatgaatcttcttacattttcgtaagtgttactcaagaagcagaaagggaagaattttttgatgaaacaagacgactttgtgaccttcggctttttcaaccctttttaaaagtaattgaaccagtaggcaaccgtgaagaaaagatcctcaatcgagaaattggttttgctatcggcatgccagtgtgtgaatttgatatggttaaagatccagaagtacaggacttccgaagaaatattctgaacgtttgtaaagaagctgtggatcttagggacctcaattcacctcatagtagagcaatgtatgtctatcctccaaatgtagaatcttcaccagaattgccaaagcacatatataataaattagataaagggcaaataatagtggtgatctgggtaatagtttctccaaataatgacaagcagaagtatactctgaaaatcaaccatgactgtgtaccagaacaagtaattgctgaagcaatcaggaaaaaaactcgaagtatgttgctatcctctgaacaactaaaactctgtgttttagaatatcagggcaagtatattttaaaagtgtgtggatgtgatgaatacttcctagaaaaatatcctctgagtcagtataagtatataagaagctgtataatgcttgggaggatgcccaatttgatgttgatggctaaagaaagcctttattctcaactgccaatggactgttttacaatgccatcttattccagacgcatttccacagctacaccatatatgaatggagaaacatctacaaaatccctttgggttataaatagtgcactcagaataaaaattctttgtgcaacctacgtgaatgtaaatattcgagacattgataagatctatgttcgaacaggtatctaccatggaggagaacccttatgtgacaatgtgaacactcaaagagtaccttgttccaatcccaggtggaatgaatggctgaattatgatatatacattcctgatcttcctcgtgctgctcgactttgcctttccatttgctctgttaaaggccgaaagggtgctaaagaggaacactgtccattggcatggggaaatataaacttgtttgattacacagacactctagtatctggaaaaatggctttgaatctttggccagtacctcatggattagaagatttgctgaaccctattggtgttactggatcaaatccaaataaagaaactccatgcttagagttggagtttgactggttcagcagtgtggtaaagttcccagatatgtcagtgattgaagagcatgccaattggtctgtatcccgagaagcaggatttagctattcccacgcaggactgagtaacagactagctagagacaatgaattaagggaaaatgacaaagaacagctcaaagcaatttctacacgagatcctctctctgaaatcactgagcaggagaaagattttctatggagtcacagacactattgtgtaactatccccgaaattctacccaaattgcttctgtctgttaaatggaattctagagatgaagtagcccagatgtattgcttggtaaaagattggcctccaatcaaacctgaacaggctatggaacttctggactgtaattacccagatcctatggttcgaggttttgctgttcggtgcttggaaaaatatttaacagatgacaaactttctcagtatttaattcagctagtacaggtcctaaaatatgaacaatatttggataacttgcttgtgagatttttactgaagaaagcattgactaatcaaaggattgggcactttttcttttggcatttaaaatctgagatgcacaataaaacagttagccagaggtttggcctgcttttggagtcctattgtcgtgcatgtgggatgtatttgaagcacctgaataggcaagtcgaggcaatggaaaagctcattaacttaactgacattctcaaacaggagaagaaggatgaaacacaaaaggtacagatgaagtttttagttgagcaaatgaggcgaccagatttcatggatgctctacagggctttctgtctcctctaaaccctgctcatcaactaggaaacctcaggcttgaagagtgtcgaattatgtcctctgcaaaaaggccactgtggttgaattgggagaacccagacatcatgtcagagttactgtttcagaacaatgagatcatctttaaaaatggggatgatttacggcaagatatgctaacacttcaaattattcgtattatggaaaatatctggcaaaatcaaggtcttgatcttcgaatgttaccttatggttgtctgtcaatcggtgactgtgtgggacttattgaggtggtgcgaaattctcacactattatgcaaattcagtgcaaaggcggcttgaaaggtgcactgcagttcaacagccacacactacatcagtggctcaaagacaagaacaaaggagaaatatatgatgcagccattgacctgtttacacgttcatgtgctggatactgtgtagctaccttcattttgggaattggagatcgtcacaatagtaacatcatggtgaaagacgatggacaactgtttcatatagattttggacactttttggatcacaagaagaaaaaatttggttataaacgagaacgtgtgccatttgttttgacacaggatttcttaatagtgattagtaaaggagcccaagaatgcacaaagacaagagaatttgagaggtttcaggagatgtgttacaaggcttatctagctattcgacagcatgccaatctcttcataaatcttttctcaatgatgcttggctctggaatgccagaactacaatcttttgatgacattgcatacattcgaaagaccctagccttagataaaactgagcaagaggctttggagtatttcatgaaacaaatgaatgatgcacatcatggtggctggacaacaaaaatggattggatcttccacacaattaaacagcatgcattgaactga

SEQ ID NO: 118 - protein, 1068 aa, Homo sapiens
MPPRPSSGELWGIHLMPPRILVECLLPNGMIVTLECLREATLITIKHELFKEARKYPLHQLLQDESSYIFVSVTQEAEREEFFDETRRLCDLRLFQPFLKVIEPVGNREEKILNREIGFAIGMPVCEFDMVKDPEVQDFRRNILNVCKEAVDLRDLNSPHSRAMYVYPPNVESSPELPKHIYNKLDKGQIIVVIWVIVSPNNDKQKYTLKINHDCVPEQVIAEAIRKKTRSMLLSSEQLKLCVLEYQGKYILKVCGCDEYFLEKYPLSQYKYIRSCIMLGRMPNLMLMAKESLYSQLPMDCFTMPSYSRRISTATPYMNGETSTKSLWVINSALRIKILCATYVNVNIRDIDKIYVRTGIYHGGEPLCDNVNTQRVPCSNPRWNEWLNYDIYIPDLPRAARLCLSICSVKGRKGAKEEHCPLAWGNINLFDYTDTLVSGKMALNLWPVPHGLEDLLNPIGVTGSNPNKETPCLELEFDWFSSVVKFPDMSVIEEHANWSVSREAGFSYSHAGLSNRLARDNELRENDKEQLKAISTRDPLSEITEQEKDFLWSHRHYCVTIPEILPKLLLSVKWNSRDEVAQMYCLVKDWPPIKPEQAMELLDCNYPDPMVRGFAVRCLEKYLTDDKLSQYLIQLVQVLKYEQYLDNLLVRFLLKKALTNQRIGHFFFWHLKSEMHNKTVSQRFGLLLESYCRACGMYLKHLNRQVEAMEKLINLTDILKQEKKDETQKVQMKFLVEQMRRPDFMDALQGFLSPLNPAHQLGNLRLEECRIMSSAKRPLWLNWENPDIMSELLFQNNEIIFKNGDDLRQDMLTLQIIRIMENIWQNQGLDLRMLPYGCLSIGDCVGLIEVVRNSHTIMQIQCKGGLKGALQFNSHTLHQWLKDKNKGEIYDAAIDLFTRSCAGYCVATFILGIGDRHNSNIMVKDDGQLFHIDFGHFLDHKKKKFGYKRERVPFVLTQDFLIVISKGAQECTKTREFERFQEMCYKAYLAIRQHANLFINLFSMMLGSGMPELQSFDDIAYIRKTLALDKTEQEALEYFMKQMNDAHHGGWTTKMDWIFHTIKQHALN

SEQ ID NO: 119 - DNA, 513 bp, Artificial Sequence
  Synthetic
gtcttcacactcgaagatttcgttggggactggcgacagacagccggctacaacctggaccaagtccttgaacagggaggtgtgtccagtttgtttcagaatctcggggtgtccgtaactccgatccaaaggattgtcctgagcggtgaaaatgggctgaagatcgacatccatgtcatcatcccgtatgaaggtctgagcggcgaccaaatgggccagatcgaaaaaatttttaaggtggtgtaccctgtggatgatcatcactttaaggtgatcctgcactatggcacactggtaatcgacggggttacgccgaacatgatcgactatttcggacggccgtatgaaggcatcgccgtgttcgacggcaaaaagatcactgtaacagggaccctgtggaacggcaacaaaattatcgacgagcgcctgatcaaccccgacggctccctgctgttccgagtaaccatcaacggagtgaccggctggcggctgtgcgaacgcattctggcgtaa

SEQ ID NO: 120 - DNA, 57 bp, Artificial Sequence
  Synthetic
gggaaataagagagaaaagaagagtaagaagaaatataagaccccggcgccgccacc

SEQ ID NO: 121 - DNA, 139 bp, Artificial Sequence
  Synthetic
taataggctggagcctcggtggcctagcttcttgccccttgggcctccccccagcccctcctccccttcctgcacccgtaccccctccataaagtaggaaacactacagtggtctttgaataaagtctgagtgggcggc

SEQ ID NO: 122 - DNA, 139 bp, Artificial Sequence
  Synthetic
ttttttttttttttttttttttttttttttttttttttttttttttttttttttttttttttttttttttttttttttttttttttttttttttttttttttttttttttttttttttttttgcacaaatattactttc

SEQ ID NO: 123 - DNA, 38 bp, Artificial Sequence
  Synthetic
taatacgactcactatagggaaataagagagaaaagaa

SEQ ID NO: 124 - DNA, 139 bp, Artificial Sequence
  Synthetic
ttttttttttttttttttttttttttttttttttttttttttttttttttttttttttttttttttttttttttttttttttttttttttttttttttttttttttttttttttttttttgccgcccactcagacttta

SEQ ID NO: 125 - DNA, 38 bp, Artificial Sequence
  Synthetic
taatacgactcactatagggtggcagctcacagctatt